European Patent Application EP 4 596 700 A1, published August 6, 2025. Title: NUCLEIC ACID CONSTRUCT AND USE THEREOF. Applicant: KANGLIN BIOTECH(HANGZHOU) CO., LTD. The sequence listing filed with the application follows.

SEQUENCE LISTING (48 sequences)

SEQ ID NO: 1 - protein, 251 aa, synthetic construct
EIVMTQSPSTLSASVGDRVIITCQASEIIHSWLAWYQQKPGKAPKLLIYLASTLASGVPSRFSGSGSGAEFTLTISSLQPDDFATYYCQNVYLASTNGANFGQGTKLTVLGGGGGSGGGGSGGGGSGGGGSEVQLVESGGGLVQPGGSLRLSCTASGFSLTDYYYMTWVRQAPGKGLEWVGFIDPDDDPYYATWAKGRFTISRDNSKNTLYLQMNSLRAEDTAVYYCAGGDHNSGWGLDIWGQGTLVTVSS

SEQ ID NO: 2 - DNA, 753 bp, synthetic construct
  source 1..753: mol_type = other DNA
gagatcgtgatgacacagagccccagcacactgtccgccagcgtgggcgacagagtgatcatcacctgtcaggcttctgaaatcatccactcttggctggcctggtaccagcagaagcccggtaaagcccctaaactgctgatctacctggcttctaccctggctagcggcgttcctagccggtttagcggatccggaagcggtgctgagttcacactgaccatttctagcctccagcctgatgacttcgccacctactattgccagaacgtgtacctcgcctctactaacggcgccaatttcggccaaggcacaaagctgaccgtgctgggcggcggcggcggcagcggcggaggcggcagcggcggaggcggcagcggcggcggcggctccgaggtgcagctggtcgagagcggcggagggctggtgcaaccaggaggctctctgagactgagctgcaccgccagcggattcagcctgacagattactattacatgacctgggtcagacaggcccctggcaagggcctggaatgggtgggatttatcgaccccgacgacgatccttactacgccacatgggccaagggcagattcaccatcagcagagataactctaagaacaccctgtacctgcagatgaacagcctgcgggccgaggacaccgccgtgtactactgcgccggcggcgaccacaattccggctggggcctggacatctggggacagggcaccctggtgaccgtgtccagc

SEQ ID NO: 3 - protein, 495 aa, synthetic construct
EVQLVESGGGLVQPGGSLRLSCAASGYDFTHYGMNWVRQAPGKGLEWVGWINTYTGEPTYAADFKRRFTFSLDTSKSTAYLQMNSLRAEDTAVYYCAKYPYYYGTSHWYFDVWGQGTLVTVSSASTKGPSVFPLAPSSKSTSGGTAALGCLVKDYFPEPVTVSWNSGALTSGVHTFPAVLQSSGLYSLSSVVTVPSSSLGTQTYICNVNHKPSNTKVDKKVEPKSCDKTHLRKRRAPVKQTLNFDLLKLAGDVESNPGPMDMRVPAQLLGLLLLWLSGARCDIQLTQSPSSLSASVGDRVTITCSASQDISNYLNWYQQKPGKAPKVLIYFTSSLHSGVPSRFSGSGSGTDFTLTISSLQPEDFATYYCQQYSTVPWTFGQGTKVEIKRTVAAPSVFIFPPSDEQLKSGTASVVCLLNNFYPREAKVQWKVDNALQSGNSQESVTEQDSKDSTYSLSSTLTLSKADYEKHKVYACEVTHQGLSSPVTKSFNRGEC

SEQ ID NO: 4 - DNA, 1485 bp, synthetic construct
  source 1..1485: mol_type = other DNA
gaggtccagctggtggagtccggcggcgggctcgtgcagccggggggctccctgcgcctgtcctgcgccgcgagcggctacgacttcacgcactacgggatgaactgggtccgccaggcgcccggcaagggcctcgagtgggtcgggtggatcaacacctacacgggcgagcccacgtacgccgcggacttcaagaggcgcttcaccttcagcctggacacgagcaagtcgacggcgtaccttcagatgaactccctgcgggcggaggacaccgcggtctactactgcgcgaagtacccgtactactacggcacctcccactggtacttcgacgtgtggggccagggcaccctcgtcacggtcagctccgcgagcacaaagggtcccagcgtgttcccgctggcccccagctcgaagagcaccagcggggggaccgccgccctcgggtgcctcgtgaaggactacttcccggaacccgtcaccgtcagctggaacagcggcgccctcacctccggcgtgcacaccttcccggccgtcctgcagagcagcgggctgtacagcctcagcagcgtcgtgactgtgccctccagctcgctagggacgcagacctacatctgcaacgtcaaccacaagccaagcaacaccaaggtcgacaagaaggtggagcccaagtcatgcgacaagacccacctgcggaaacggcgggcccccgtcaagcagaccctgaacttcgacctgctcaagctagcgggcgacgtagagagcaacccgggccccatggacatgcgggtccccgcccagctgctcgggctgctcctactctggctcagcggggcgcgttgcgacatccagctcacgcagagccccagtagcctgagcgccagcgtgggcgaccgggtgaccatcacgtgctccgccagccaggacatcagcaactacctcaactggtaccagcagaagcccgggaaggccccgaaggtgctcatctacttcacgagcagcctgcacagcggggtgccctcccgcttcagcgggagcgggtccgggacagacttcacgctcaccatctccagcctgcagcccgaggacttcgcgacctactactgccagcagtacagcacggtgccctggaccttcggccaggggaccaaggtcgagatcaagcgcacggtggcggcgcccagcgtcttcatcttccccccgagcgacgagcagctcaagagcggcaccgcgagcgtcgtgtgccttctcaacaacttctacccccgggaggcgaaggtccagtggaaggtggacaacgccctccagtccgggaacagccaggagagcgtgaccgagcaggacagcaaggacagcacgtacagcctcagctccacgctcaccctctccaaggccgactacgagaagcacaaggtgtacgcgtgcgaggtcacccaccaggggctgtcgagcccggtgacgaagagcttcaaccgaggggagtgc

SEQ ID NO: 5 - protein, 205 aa, synthetic construct
SDTGRPFVEMYSEIPEIIHMTEGRELVIPCRVTSPNITVTLKKFPLDTLIPDGKRIIWDSRKGFIISNATYKEIGLLTCEATVNGHLYKTNYLTHRQTNTIIDVVLSPSHGIELSVGEKLVLNCTARTELNVGIDFNWEYPSSKHQHKKLVNRDLKTQSGSEMKKFLSTLTIDGVTRSDQGLYTCAASSGLMTKKNSTFVRVHEK

SEQ ID NO: 6 - DNA, 615 bp, synthetic construct
  source 1..615: mol_type = other DNA
tccgacacaggcagacccttcgtggagatgtattctgagatccctgagatcatccacatgaccgagggcagggagctggtcatcccatgtcgcgtgacaagccccaacatcaccgtgacactgaagaagttccctctggacaccctgatcccagatggcaagcggatcatctgggacagcagaaagggctttatcatctccaatgccacatacaaggagatcggcctgctgacctgcgaggccacagtgaacggccacctgtacaagaccaattatctgacacacagacagaccaacacaatcatcgatgtggtgctgagcccatcccacggcatcgagctgtccgtgggcgagaagctggtgctgaattgtaccgccaggacagagctgaacgtgggcatcgacttcaattgggagtacccctctagcaagcaccagcacaagaagctggtgaacagggatctgaagacccagtctggcagcgagatgaagaagtttctgagcaccctgacaatcgacggagtgacccgctccgatcagggactgtatacatgcgccgcctcctctggcctgatgaccaagaagaattccacattcgtgcgggtgcacgagaag

SEQ ID NO: 7 - protein, 757 aa, synthetic construct
EIVMTQSPSTLSASVGDRVIITCQASEIIHSWLAWYQQKPGKAPKLLIYLASTLASGVPSRFSGSGSGAEFTLTISSLQPDDFATYYCQNVYLASTNGANFGQGTKLTVLGGGGGSGGGGSGGGGSGGGGSEVQLVESGGGLVQPGGSLRLSCTASGFSLTDYYYMTWVRQAPGKGLEWVGFIDPDDDPYYATWAKGRFTISRDNSKNTLYLQMNSLRAEDTAVYYCAGGDHNSGWGLDIWGQGTLVTVSSGGGGSGGGGSGGGGSGGGGSGGGGSDIQLTQSPSSLSASVGDRVTITCSASQDISNYLNWYQQKPGKAPKVLIYFTSSLHSGVPSRFSGSGSGTDFTLTISSLQPEDFATYYCQQYSTVPWTFGQGTKVEIKGGGGSGGGGSGGGGSGGGGSEVQLVESGGGLVQPGGSLRLSCAASGYDFTHYGMNWVRQAPGKGLEWVGWINTYTGEPTYAADFKRRFTFSLDTSKSTAYLQMNSLRAEDTAVYYCAKYPYYYGTSHWYFDVWGQGTLVTVSSEPKSCDKTHTCPPCPAPELLGGPSVFLFPPKPKDTLMISRTPEVTCVVVDVSHEDPEVKFNWYVDGVEVHNAKTKPREEQYNSTYRVVSVLTVLHQDWLNGKEYKCKVSNKALPAPIEKTISKAKGQPREPQVYTLPPSRDELTKNQVSLTCLVKGFYPSDIAVEWESNGQPENNYKTTPPVLDSDGSFFLYSKLTVDKSRWQQGNVFSCSVMHEALHNHYTQKSLSLSPG

SEQ ID NO: 8 - DNA, 2271 bp, synthetic construct
  source 1..2271: mol_type = other DNA
gagatcgtgatgacccagagccctagcacactgagcgcctctgtgggagatagagtgatcatcacctgtcaggcctctgagatcatccacagctggctggcttggtaccagcaaaagcctgggaaggcccctaaactgctgatctatctcgctagcacactggcctctggagtccccagccggtttagcggaagcggctctggcgccgaattcaccctgacaatcagcagcctgcaacccgatgactttgccacatactactgtcagaacgtgtacctggctagcaccaacggcgccaacttcggccagggcacaaagctgaccgtgcttggaggcggcggcggctccggcggaggcggaagcggcggcggcggcagcggcgggggcggcagcgaggtgcagctggtggagtcgggcggcggcctggtgcagccaggaggttctctgaggctgagctgcaccgcaagcggcttcagcctgaccgactactactatatgacatgggtcagacaggcccctggaaagggcctggaatgggtcggatttatcgaccctgacgacgatccttactacgccacttgggccaagggcagatttaccatttccagagataactctaagaacaccctgtacctgcaaatgaacagcctgcgcgccgaggatacagccgtgtactactgcgcaggcggcgaccataattcaggatggggcctggatatctggggccagggcacgctggtgaccgtgtcctccggcggaggaggctctggcggaggcggcagcggcggcggcggctccggcggcggcggcagcggcggtggcggcagcgacatccagctgacacagtccccaagcagcctgagcgcttctgtgggcgacagagtgaccatcacatgcagcgcctctcaggacatcagtaactacctgaactggtaccagcagaaacctggtaaggcccccaaggtgctgatctacttcaccagcagcctgcactctggcgtgcctagcagattcagcggcagcggatctggcacagacttcaccctgaccattagctccctgcagcctgaggacttcgccacatactactgccagcagtactccaccgttccctggaccttcggccaggggaccaaggtggagatcaaggggggcggcggcagcggaggaggcggaagcggcgggggcggatctggaggaggaggtagcgaagtgcagctggtggaaagcgggggcggcctggtgcaacctggcggcagcctcagactgagctgcgccgctagcggatatgatttcacacactacggcatgaattgggtgcggcaggctcctggcaagggcctggaatgggtgggctggatcaatacctacaccggcgagcctacatacgccgccgacttcaagcggagattcaccttctctctggacaccagcaaaagcaccgcctacctgcagatgaacagtctgcgggccgaggacaccgccgtgtactactgcgccaagtacccctactattacggcaccagccactggtacttcgacgtgtgggggcagggcaccctggtgacagtgagttcagagcctaaatcttgcgacaagacccacacatgcccaccttgtccagcaccagagctgctgggaggaccaagcgtgttcctgtttccacccaagcccaaggataccctgatgatctccaggaccccagaggtgacatgcgtggtggtggacgtgtctcacgaggatcctgaggtgaagtttaactggtacgtggacggcgtggaggtgcacaatgccaagaccaagcctcgggaggagcagtacaattccacctatagagtggtgtctgtgctgacagtgctgcaccaggattggctgaacggcaaggagtataagtgcaaggtgagcaataaggccctgcctgccccaatcgagaagaccatctccaaggcaaagggacagccaagggagcctcaggtgtacacactgcctccatctcgcgacgagctgaccaagaaccaggtgagcctgacatgtctggtgaagggcttctatccttccgatatcgccgtggagtgggagtctaatggccagccagagaacaattacaagaccacaccccctgtgctggacagcgatggctccttctttctgtattctaagctgaccgtggataagagccggtggcagcagggcaacgtgttttcctgctctgtgatgcacgaggccctgcacaatcactacacccagaagagcctgtccctgtctcccggc

SEQ ID NO: 9 - protein, 526 aa, synthetic construct
EIVMTQSPSTLSASVGDRVIITCQASEIIHSWLAWYQQKPGKAPKLLIYLASTLASGVPSRFSGSGSGAEFTLTISSLQPDDFATYYCQNVYLASTNGANFGQGTKLTVLGGGGGSGGGGSGGGGSGGGGSEVQLVESGGGLVQPGGSLRLSCTASGFSLTDYYYMTWVRQAPGKGLEWVGFIDPDDDPYYATWAKGRFTISRDNSKNTLYLQMNSLRAEDTAVYYCAGGDHNSGWGLDIWGQGTLVTVSSGGGGSGGGGSGGGGSGGGGSGGGGSDIQLTQSPSSLSASVGDRVTITCSASQDISNYLNWYQQKPGKAPKVLIYFTSSLHSGVPSRFSGSGSGTDFTLTISSLQPEDFATYYCQQYSTVPWTFGQGTKVEIKGGGGSGGGGSGGGGSGGGGSEVQLVESGGGLVQPGGSLRLSCAASGYDFTHYGMNWVRQAPGKGLEWVGWINTYTGEPTYAADFKRRFTFSLDTSKSTAYLQMNSLRAEDTAVYYCAKYPYYYGTSHWYFDVWGQGTLVTVSS

SEQ ID NO: 10 - protein, 1578 aa, synthetic construct
GAGATCGTGATGACCCAGAGCCCTAGCACACTGAGCGCCTCTGTGGGAGATAGAGTGATCATCACCTGTCAGGCCTCTGAGATCATCCACAGCTGGCTGGCTTGGTACCAGCAAAAGCCTGGGAAGGCCCCTAAACTGCTGATCTATCTCGCTAGCACACTGGCCTCTGGAGTCCCCAGCCGGTTTAGCGGAAGCGGCTCTGGCGCCGAATTCACCCTGACAATCAGCAGCCTGCAACCCGATGACTTTGCCACATACTACTGTCAGAACGTGTACCTGGCTAGCACCAACGGCGCCAACTTCGGCCAGGGCACAAAGCTGACCGTGCTTGGAGGCGGCGGCGGCTCCGGCGGAGGCGGAAGCGGCGGCGGCGGCAGCGGCGGGGGCGGCAGCGAGGTGCAGCTGGTGGAGTCGGGCGGCGGCCTGGTGCAGCCAGGAGGTTCTCTGAGGCTGAGCTGCACCGCAAGCGGCTTCAGCCTGACCGACTACTACTATATGACATGGGTCAGACAGGCCCCTGGAAAGGGCCTGGAATGGGTCGGATTTATCGACCCTGACGACGATCCTTACTACGCCACTTGGGCCAAGGGCAGATTTACCATTTCCAGAGATAACTCTAAGAACACCCTGTACCTGCAAATGAACAGCCTGCGCGCCGAGGATACAGCCGTGTACTACTGCGCAGGCGGCGACCATAATTCAGGATGGGGCCTGGATATCTGGGGCCAGGGCACGCTGGTGACCGTGTCCTCCGGCGGAGGAGGCTCTGGCGGAGGCGGCAGCGGCGGCGGCGGCTCCGGCGGCGGCGGCAGCGGCGGTGGCGGCAGCGACATCCAGCTGACACAGTCCCCAAGCAGCCTGAGCGCTTCTGTGGGCGACAGAGTGACCATCACATGCAGCGCCTCTCAGGACATCAGTAACTACCTGAACTGGTACCAGCAGAAACCTGGTAAGGCCCCCAAGGTGCTGATCTACTTCACCAGCAGCCTGCACTCTGGCGTGCCTAGCAGATTCAGCGGCAGCGGATCTGGCACAGACTTCACCCTGACCATTAGCTCCCTGCAGCCTGAGGACTTCGCCACATACTACTGCCAGCAGTACTCCACCGTTCCCTGGACCTTCGGCCAGGGGACCAAGGTGGAGATCAAGGGGGGCGGCGGCAGCGGAGGAGGCGGAAGCGGCGGGGGCGGATCTGGAGGAGGAGGTAGCGAAGTGCAGCTGGTGGAAAGCGGGGGCGGCCTGGTGCAACCTGGCGGCAGCCTCAGACTGAGCTGCGCCGCTAGCGGATATGATTTCACACACTACGGCATGAATTGGGTGCGGCAGGCTCCTGGCAAGGGCCTGGAATGGGTGGGCTGGATCAATACCTACACCGGCGAGCCTACATACGCCGCCGACTTCAAGCGGAGATTCACCTTCTCTCTGGACACCAGCAAAAGCACCGCCTACCTGCAGATGAACAGTCTGCGGGCCGAGGACACCGCCGTGTACTACTGCGCCAAGTACCCCTACTATTACGGCACCAGCCACTGGTACTTCGACGTGTGGGGGCAGGGCACCCTGGTGACAGTGAGTTCA

SEQ ID NO: 11 - protein, 711 aa, synthetic construct
SDTGRPFVEMYSEIPEIIHMTEGRELVIPCRVTSPNITVTLKKFPLDTLIPDGKRIIWDSRKGFIISNATYKEIGLLTCEATVNGHLYKTNYLTHRQTNTIIDVVLSPSHGIELSVGEKLVLNCTARTELNVGIDFNWEYPSSKHQHKKLVNRDLKTQSGSEMKKFLSTLTIDGVTRSDQGLYTCAASSGLMTKKNSTFVRVHEKGGGGSGGGGSGGGGSGGGGSGGGGSDIQLTQSPSSLSASVGDRVTITCSASQDISNYLNWYQQKPGKAPKVLIYFTSSLHSGVPSRFSGSGSGTDFTLTISSLQPEDFATYYCQQYSTVPWTFGQGTKVEIKGGGGSGGGGSGGGGSGGGGSEVQLVESGGGLVQPGGSLRLSCAASGYDFTHYGMNWVRQAPGKGLEWVGWINTYTGEPTYAADFKRRFTFSLDTSKSTAYLQMNSLRAEDTAVYYCAKYPYYYGTSHWYFDVWGQGTLVTVSSEPKSCDKTHTCPPCPAPELLGGPSVFLFPPKPKDTLMISRTPEVTCVVVDVSHEDPEVKFNWYVDGVEVHNAKTKPREEQYNSTYRVVSVLTVLHQDWLNGKEYKCKVSNKALPAPIEKTISKAKGQPREPQVYTLPPSRDELTKNQVSLTCLVKGFYPSDIAVEWESNGQPENNYKTTPPVLDSDGSFFLYSKLTVDKSRWQQGNVFSCSVMHEALHNHYTQKSLSLSPG

SEQ ID NO: 12 - DNA, 2133 bp, synthetic construct
  source 1..2133: mol_type = other DNA
agcgacaccggcagacctttcgtggaaatgtacagcgagatcccagagattatccacatgaccgagggccgggaactggtgatcccctgcagagttaccagcccaaacatcaccgtgaccctcaagaagttccccctggatacactgatccctgacggcaaaagaatcatctgggacagcagaaagggcttcatcatcagcaacgccacctacaaggaaatcggcctgctgacatgcgaggccaccgtgaacggccacctgtacaagaccaactacctgacccatagacagaccaatacaatcatcgatgtggtgctgagcccttcccacggaatcgagctgtccgtgggagaaaagctggtgctaaattgcaccgccagaacagaactgaacgtgggcatcgacttcaactgggagtacccttctagcaagcaccagcacaagaagctggtcaaccgggacctcaagacacagagcggctccgagatgaaaaaatttctgtctacactgacaatcgacggcgtcacaagatccgatcagggactgtacacctgtgccgctagcagcggactgatgaccaagaagaactctaccttcgtgcgggtgcacgagaagggcggcggcggctctggcggcggcggcagcggcggaggcggctccggcggcggcggcagcggcggcggaggaagcgacatccagctgacacaaagccccagcagcctgtcagcctctgtgggcgaccgggtgaccatcacatgcagcgccagccaggatatcagcaattaccttaactggtatcagcagaagcccggcaaggcccctaaggtgctgatctacttcaccagtagcctgcacagcggggtgccttctagatttagcggaagcggaagcgggactgactttaccctgaccatctcttctctgcagcctgaggattttgccacatactactgtcagcaatacagcaccgtcccttggaccttcggccagggcaccaaggtggaaataaagggcggcggcggctctggaggcggtggcagcgggggcggcggcagcggcggaggcggatccgaggtgcagctggttgaaagcggcggcggcctggtgcagcccggcggaagcctgcggctgagctgtgctgctagcggctacgacttcacccactacggcatgaactgggtgcgccaggctcctggaaaaggcctcgaatgggtcggatggatcaacacatacaccggcgagcctacatacgccgccgatttcaagcgaagattcaccttctctctggacactagcaagtccaccgcctacctgcaaatgaacagcctgagggccgaggatacagccgtgtactattgcgcaaagtacccatactattacggcaccagccactggtacttcgacgtgtggggccagggcaccctggtgaccgtgtcttctgagcctaaatcttgcgacaagacccacacatgcccaccttgtccagcaccagagctgctgggaggaccaagcgtgttcctgtttccacccaagcccaaggataccctgatgatctccaggaccccagaggtgacatgcgtggtggtggacgtgtctcacgaggatcctgaggtgaagtttaactggtacgtggacggcgtggaggtgcacaatgccaagaccaagcctcgggaggagcagtacaattccacctatagagtggtgtctgtgctgacagtgctgcaccaggattggctgaacggcaaggagtataagtgcaaggtgagcaataaggccctgcctgccccaatcgagaagaccatctccaaggcaaagggacagccaagggagcctcaggtgtacacactgcctccatctcgcgacgagctgaccaagaaccaggtgagcctgacatgtctggtgaagggcttctatccttccgatatcgccgtggagtgggagtctaatggccagccagagaacaattacaagaccacaccccctgtgctggacagcgatggctccttctttctgtattctaagctgaccgtggataagagccggtggcagcagggcaacgtgttttcctgctctgtgatgcacgaggccctgcacaatcactacacccagaagagcctgtccctgtctcccggc

SEQ ID NO: 13 - protein, 480 aa, synthetic construct
SDTGRPFVEMYSEIPEIIHMTEGRELVIPCRVTSPNITVTLKKFPLDTLIPDGKRIIWDSRKGFIISNATYKEIGLLTCEATVNGHLYKTNYLTHRQTNTIIDVVLSPSHGIELSVGEKLVLNCTARTELNVGIDFNWEYPSSKHQHKKLVNRDLKTQSGSEMKKFLSTLTIDGVTRSDQGLYTCAASSGLMTKKNSTFVRVHEKGGGGSGGGGSGGGGSGGGGSGGGGSDIQLTQSPSSLSASVGDRVTITCSASQDISNYLNWYQQKPGKAPKVLIYFTSSLHSGVPSRFSGSGSGTDFTLTISSLQPEDFATYYCQQYSTVPWTFGQGTKVEIKGGGGSGGGGSGGGGSGGGGSEVQLVESGGGLVQPGGSLRLSCAASGYDFTHYGMNWVRQAPGKGLEWVGWINTYTGEPTYAADFKRRFTFSLDTSKSTAYLQMNSLRAEDTAVYYCAKYPYYYGTSHWYFDVWGQGTLVTVSS

SEQ ID NO: 14 - DNA, 1440 bp, synthetic construct
  source 1..1440: mol_type = other DNA
agcgacaccggcagacctttcgtggaaatgtacagcgagatcccagagattatccacatgaccgagggccgggaactggtgatcccctgcagagttaccagcccaaacatcaccgtgaccctcaagaagttccccctggatacactgatccctgacggcaaaagaatcatctgggacagcagaaagggcttcatcatcagcaacgccacctacaaggaaatcggcctgctgacatgcgaggccaccgtgaacggccacctgtacaagaccaactacctgacccatagacagaccaatacaatcatcgatgtggtgctgagcccttcccacggaatcgagctgtccgtgggagaaaagctggtgctaaattgcaccgccagaacagaactgaacgtgggcatcgacttcaactgggagtacccttctagcaagcaccagcacaagaagctggtcaaccgggacctcaagacacagagcggctccgagatgaaaaaatttctgtctacactgacgatcgacggcgtcacaagatccgatcagggactgtacacctgtgccgctagcagcggactgatgaccaagaagaactctaccttcgtgcgggtgcacgagaagggcggcggcggctctggcggcggcggcagcggcggaggcggctccggcggcggcggcagcggcggcggaggaagcgacatccagctgacacaaagccccagcagcctgtcagcctctgtgggcgaccgggtgaccatcacatgcagcgccagccaggatatcagcaattaccttaactggtatcagcagaagcccggcaaggcccctaaggtgctgatctacttcaccagtagcctgcacagcggggtgccttctagatttagcggaagcggaagcgggactgactttaccctgaccatctcttctctgcagcctgaggattttgccacatactactgtcagcaatacagcaccgtcccttggaccttcggccagggcaccaaggtggaaataaagggcggcggcggctctggaggcggtggcagcgggggcggcggcagcggcggaggcggatccgaggtgcagctggttgaaagcggcggcggcctggtgcagcccggcggaagcctgcggctgagctgtgctgctagcggctacgacttcacccactacggcatgaactgggtgcgccaggctcctggaaaaggcctcgaatgggtcggatggatcaacacatacaccggcgagcctacatacgccgccgatttcaagcgaagattcaccttctctctggacactagcaagtccaccgcctacctgcaaatgaacagcctgagggccgaggatacagccgtgtactattgcgcaaagtacccatactattacggcaccagccactggtacttcgacgtgtggggccagggcaccctggtgaccgtgtcttct

SEQ ID NO: 15 - protein, 987 aa, synthetic construct
SDTGRPFVEMYSEIPEIIHMTEGRELVIPCRVTSPNITVTLKKFPLDTLIPDGKRIIWDSRKGFIISNATYKEIGLLTCEATVNGHLYKTNYLTHRQTNTIIDVVLSPSHGIELSVGEKLVLNCTARTELNVGIDFNWEYPSSKHQHKKLVNRDLKTQSGSEMKKFLSTLTIDGVTRSDQGLYTCAASSGLMTKKNSTFVRVHEKGGGGSGGGGSGGGGSGGGGSGGGGSEIVMTQSPSTLSASVGDRVIITCQASEIIHSWLAWYQQKPGKAPKLLIYLASTLASGVPSRFSGSGSGAEFTLTISSLQPDDFATYYCQNVYLASTNGANFGQGTKLTVLGGGGGSGGGGSGGGGSGGGGSEVQLVESGGGLVQPGGSLRLSCTASGFSLTDYYYMTWVRQAPGKGLEWVGFIDPDDDPYYATWAKGRFTISRDNSKNTLYLQMNSLRAEDTAVYYCAGGDHNSGWGLDIWGQGTLVTVSSGGGGSGGGGSGGGGSGGGGSGGGGSDIQLTQSPSSLSASVGDRVTITCSASQDISNYLNWYQQKPGKAPKVLIYFTSSLHSGVPSRFSGSGSGTDFTLTISSLQPEDFATYYCQQYSTVPWTFGQGTKVEIKGGGGSGGGGSGGGGSGGGGSEVQLVESGGGLVQPGGSLRLSCAASGYDFTHYGMNWVRQAPGKGLEWVGWINTYTGEPTYAADFKRRFTFSLDTSKSTAYLQMNSLRAEDTAVYYCAKYPYYYGTSHWYFDVWGQGTLVTVSSEPKSCDKTHTCPPCPAPELLGGPSVFLFPPKPKDTLMISRTPEVTCVVVDVSHEDPEVKFNWYVDGVEVHNAKTKPREEQYNSTYRVVSVLTVLHQDWLNGKEYKCKVSNKALPAPIEKTISKAKGQPREPQVYTLPPSRDELTKNQVSLTCLVKGFYPSDIAVEWESNGQPENNYKTTPPVLDSDGSFFLYSKLTVDKSRWQQGNVFSCSVMHEALHNHYTQKSLSLSPG

SEQ ID NO: 16 - DNA, 2961 bp, synthetic construct
  source 1..2961: mol_type = other DNA
agcgacaccggccggcctttcgtggaaatgtacagcgagatccccgagatcatccacatgaccgagggcagagagctggtgatcccctgccgggtgaccagccctaacatcaccgtgaccctgaagaaattccccctggacacactgatccccgatggaaaaagaatcatctgggacagcagaaagggcttcatcatttctaatgccacatacaaggaaatcggcctgctgacttgtgaagccaccgtgaacggccacctgtacaagaccaactacctgactcatagacaaacaaacacaatcatcgacgtggtgctgagcccttctcatggcatcgagctctctgtgggcgagaagctggtgctgaattgcaccgctcgcaccgagctgaacgtgggaatcgacttcaactgggagtacccttcttctaagcaccagcacaagaagctggtgaaccgggacctgaagacccagagcggcagcgaaatgaaaaagttcctgtccacactgaccattgacggcgtgacaagaagcgaccagggcctgtatacatgtgccgcctcttctgggctgatgaccaagaagaacagcaccttcgtgcgggtgcacgagaagggcggcggtggctcaggaggtggcggcagcggcggcggcggatcgggcgggggcggctctggaggcggcggtagcgagatcgtgatgacccagagccccagcaccctgtccgccagcgtgggcgacagagtgatcatcacttgccaggcctccgaaatcatccacagctggctggcttggtaccagcagaaacctggcaaggctccaaagctgctgatctacctggccagcaccctcgctagcggcgttccttccagattcagcggcagcggctccggagctgaattcaccctgaccatcagctctctgcagcctgacgacttcgccacatactactgtcagaacgtgtacctggcttctacaaacggcgccaatttcggccagggcacaaaactgacagtgctgggcggcggtggaggatcgggaggcggcggctctggaggcggcggcagcggcggcggcggctctgaagtgcaactggttgagagcggcgggggcctggtgcagcccggtggctccctgagactgagctgcaccgccagcggatttagcctgacagattactattacatgacatgggtcagacaggccccaggcaagggcctggaatgggtcggcttcatcgatcctgatgatgacccctactacgccacttgggccaaggggaggttcaccatttctagagataacagcaagaacaccctgtacctgcagatgaacagcctgagagccgaggacaccgccgtgtactactgcgccggcggagatcacaacagcggctggggcctggatatctggggacagggcaccctggtgaccgtgtctagcggcggcggcggcagcggcggcggcggcagcggcggcggcggctctggcggcggcggaagcggaggtggaggttccgatatccagctgacacagagtcctagctcccttagcgctagcgtgggcgacagagtgaccatcacctgcagcgccagccaggacattagcaattacctgaactggtaccagcaaaagcctggcaaagcccctaaggtactgatctacttcaccagcagcctgcactctggggtgccttcccggttcagcggatctggctctggtaccgattttaccctgacaatctcctctctgcagccagaggattttgccacctactactgccagcagtacagcaccgtgccctggacatttggacaaggaaccaaggtggaaatcaagggaggcggcggaagcggcggcggcggtagcggcggtggcggtagcggcggtggaggcagcgaggtgcagctggtggaaagcggcggaggcctcgtgcaacctggcggctccctgagactgagttgtgccgcttccggctacgacttcacacactacggcatgaactgggtgcggcaggctccaggcaagggcctggagtgggtgggatggatcaacacctacaccggagaacctacatatgctgccgactttaagcgtaggttcaccttcagcctggacaccagcaagagcacagcctacctgcagatgaattctctgcgggccgaggacaccgccgtgtactactgcgccaagtacccctactactatggcaccagccactggtatttcgacgtgtggggccagggcacactggttaccgtcagctctgagcctaaatcttgcgacaagacccacacatgcccaccttgtccagcaccagagctgctgggaggaccaagcgtgttcctgtttccacccaagcccaaggataccctgatgatctccaggaccccagaggtgacatgcgtggtggtggacgtgtctcacgaggatcctgaggtgaagtttaactggtacgtggacggcgtggaggtgcacaatgccaagaccaagcctcgggaggagcagtacaattccacctatagagtggtgtctgtgctgacagtgctgcaccaggattggctgaacggcaaggagtataagtgcaaggtgagcaataaggccctgcctgccccaatcgagaagaccatctccaaggcaaagggacagccaagggagcctcaggtgtacacactgcctccatctcgcgacgagctgaccaagaaccaggtgagcctgacatgtctggtgaagggcttctatccttccgatatcgccgtggagtgggagtctaatggccagccagagaacaattacaagaccacaccccctgtgctggacagcgatggctccttctttctgtattctaagctgaccgtggataagagccggtggcagcagggcaacgtgttttcctgctctgtgatgcacgaggccctgcacaatcactacacccagaagagcctgtccctgtctcccggc

SEQ ID NO: 17 - protein, 756 aa, synthetic construct
SDTGRPFVEMYSEIPEIIHMTEGRELVIPCRVTSPNITVTLKKFPLDTLIPDGKRIIWDSRKGFIISNATYKEIGLLTCEATVNGHLYKTNYLTHRQTNTIIDVVLSPSHGIELSVGEKLVLNCTARTELNVGIDFNWEYPSSKHQHKKLVNRDLKTQSGSEMKKFLSTLTIDGVTRSDQGLYTCAASSGLMTKKNSTFVRVHEKGGGGSGGGGSGGGGSGGGGSGGGGSEIVMTQSPSTLSASVGDRVIITCQASEIIHSWLAWYQQKPGKAPKLLIYLASTLASGVPSRFSGSGSGAEFTLTISSLQPDDFATYYCQNVYLASTNGANFGQGTKLTVLGGGGGSGGGGSGGGGSGGGGSEVQLVESGGGLVQPGGSLRLSCTASGFSLTDYYYMTWVRQAPGKGLEWVGFIDPDDDPYYATWAKGRFTISRDNSKNTLYLQMNSLRAEDTAVYYCAGGDHNSGWGLDIWGQGTLVTVSSGGGGSGGGGSGGGGSGGGGSGGGGSDIQLTQSPSSLSASVGDRVTITCSASQDISNYLNWYQQKPGKAPKVLIYFTSSLHSGVPSRFSGSGSGTDFTLTISSLQPEDFATYYCQQYSTVPWTFGQGTKVEIKGGGGSGGGGSGGGGSGGGGSEVQLVESGGGLVQPGGSLRLSCAASGYDFTHYGMNWVRQAPGKGLEWVGWINTYTGEPTYAADFKRRFTFSLDTSKSTAYLQMNSLRAEDTAVYYCAKYPYYYGTSHWYFDVWGQGTLVTVSS

SEQ ID NO: 18 - DNA, 2268 bp, synthetic construct
  source 1..2268: mol_type = other DNA
agcgacaccggccggcctttcgtggaaatgtacagcgagatccccgagatcatccacatgaccgagggcagagagctggtgatcccctgccgggtgaccagccctaacatcaccgtgaccctgaagaaattccccctggacacactgatccccgatggaaaaagaatcatctgggacagcagaaagggcttcatcatttctaatgccacatacaaggaaatcggcctgctgacttgtgaagccaccgtgaacggccacctgtacaagaccaactacctgactcatagacaaacaaacacaatcatcgacgtggtgctgagcccttctcatggcatcgagctctctgtgggcgagaagctggtgctgaattgcaccgctcgcaccgagctgaacgtgggaatcgacttcaactgggagtacccttcttctaagcaccagcacaagaagctggtgaaccgggacctgaagacccagagcggcagcgaaatgaaaaagttcctgtccacactgaccattgacggcgtgacaagaagcgaccagggcctgtatacatgtgccgcctcttctgggctgatgaccaagaagaacagcaccttcgtgcgggtgcacgagaagggcggcggtggctcaggaggtggcggcagcggcggcggcggatcgggcgggggcggctctggaggcggcggtagcgagatcgtgatgacccagagccccagcaccctgtccgccagcgtgggcgacagagtgatcatcacttgccaggcctccgaaatcatccacagctggctggcttggtaccagcagaaacctggcaaggctccaaagctgctgatctacctggccagcaccctcgctagcggcgttccttccagattcagcggcagcggctccggagctgaattcaccctgaccatcagctctctgcagcctgacgacttcgccacatactactgtcagaacgtgtacctggcttctacaaacggcgccaatttcggccagggcacaaaactgacagtgctgggcggcggtggaggatcgggaggcggcggctctggaggcggcggcagcggcggcggcggctctgaagtgcaactggttgagagcggcgggggcctggtgcagcccggtggctccctgagactgagctgcaccgccagcggatttagcctgacagattactattacatgacatgggtcagacaggccccaggcaagggcctggaatgggtcggcttcatcgatcctgatgatgacccctactacgccacttgggccaaggggaggttcaccatttctagagataacagcaagaacaccctgtacctgcagatgaacagcctgagagccgaggacaccgccgtgtactactgcgccggcggagatcacaacagcggctggggcctggatatctggggacagggcaccctggtgaccgtgtctagcggcggcggcggcagcggcggcggcggcagcggcggcggcggctctggcggcggcggaagcggaggtggaggttccgatatccagctgacacagagtcctagctcccttagcgctagcgtgggcgacagagtgaccatcacctgcagcgccagccaggacattagcaattacctgaactggtaccagcaaaagcctggcaaagcccctaaggtactgatctacttcaccagcagcctgcactctggggtgccttcccggttcagcggatctggctctggtaccgattttaccctgacaatctcctctctgcagccagaggattttgccacctactactgccagcagtacagcaccgtgccctggacatttggacaaggaaccaaggtggaaatcaagggaggcggcggaagcggcggcggcggtagcggcggtggcggtagcggcggtggaggcagcgaggtgcagctggtggaaagcggcggaggcctcgtgcaacctggcggctccctgagactgagttgtgccgcttccggctacgacttcacacactacggcatgaactgggtgcggcaggctccaggcaagggcctggagtgggtgggatggatcaacacctacaccggagaacctacatatgctgccgactttaagcgtaggttcaccttcagcctggacaccagcaagagcacagcctacctgcagatgaattctctgcgggccgaggacaccgccgtgtactactgcgccaagtacccctactactatggcaccagccactggtatttcgacgtgtggggccagggcacactggttaccgtcagctct

SEQ ID NO: 19 - protein, 481 aa, synthetic construct
SDTGRPFVEMYSEIPEIIHMTEGRELVIPCRVTSPNITVTLKKFPLDTLIPDGKRIIWDSRKGFIISNATYKEIGLLTCEATVNGHLYKTNYLTHRQTNTIIDVVLSPSHGIELSVGEKLVLNCTARTELNVGIDFNWEYPSSKHQHKKLVNRDLKTQSGSEMKKFLSTLTIDGVTRSDQGLYTCAASSGLMTKKNSTFVRVHEKGGGGSGGGGSGGGGSGGGGSGGGGSEIVMTQSPSTLSASVGDRVIITCQASEIIHSWLAWYQQKPGKAPKLLIYLASTLASGVPSRFSGSGSGAEFTLTISSLQPDDFATYYCQNVYLASTNGANFGQGTKLTVLGGGGGSGGGGSGGGGSGGGGSEVQLVESGGGLVQPGGSLRLSCTASGFSLTDYYYMTWVRQAPGKGLEWVGFIDPDDDPYYATWAKGRFTISRDNSKNTLYLQMNSLRAEDTAVYYCAGGDHNSGWGLDIWGQGTLVTVSS

SEQ ID NO: 20 - DNA, 1443 bp, synthetic construct
  source 1..1443: mol_type = other DNA
agcgacaccggccggcctttcgtggaaatgtacagcgagatccccgagatcatccacatgaccgagggcagagagctggtgatcccctgccgggtgaccagccctaacatcaccgtgaccctgaagaaattccccctggacacactgatccccgatggaaaaagaatcatctgggacagcagaaagggcttcatcatttctaatgccacatacaaggaaatcggcctgctgacttgtgaagccaccgtgaacggccacctgtacaagaccaactacctgactcatagacaaacaaacacaatcatcgacgtggtgctgagcccttctcatggcatcgagctctctgtgggcgagaagctggtgctgaattgcaccgctcgcaccgagctgaacgtgggaatcgacttcaactgggagtacccttcttctaagcaccagcacaagaagctggtgaaccgggacctgaagacccagagcggcagcgaaatgaaaaagttcctgtccacactgaccattgacggcgtgacaagaagcgaccagggcctgtatacatgtgccgcctcttctgggctgatgaccaagaagaacagcaccttcgtgcgggtgcacgagaagggcggcggtggctcaggaggtggcggcagcggcggcggcggatcgggcgggggcggctctggaggcggcggtagcgagatcgtgatgacccagagccccagcaccctgtccgccagcgtgggcgacagagtgatcatcacttgccaggcctccgaaatcatccacagctggctggcttggtaccagcagaaacctggcaaggctccaaagctgctgatctacctggccagcaccctcgctagcggcgttccttccagattcagcggcagcggctccggagctgaattcaccctgaccatcagctctctgcagcctgacgacttcgccacatactactgtcagaacgtgtacctggcttctacaaacggcgccaatttcggccagggcacaaaactgacagtgctgggcggcggtggaggatcgggaggcggcggctctggaggcggcggcagcggcggcggcggctctgaagtgcaactggttgagagcggcgggggcctggtgcagcccggtggctccctgagactgagctgcaccgccagcggatttagcctgacagattactattacatgacatgggtcagacaggccccaggcaagggcctggaatgggtcggcttcatcgatcctgatgatgacccctactacgccacttgggccaaggggaggttcaccatttctagagataacagcaagaacaccctgtacctgcagatgaacagcctgagagccgaggacaccgccgtgtactactgcgccggcggagatcacaacagcggctggggcctggatatctggggacagggcaccctggtgaccgtgtctagc

SEQ ID NO: 21 - protein, 481 aa, synthetic construct
EIVMTQSPSTLSASVGDRVIITCQASEIIHSWLAWYQQKPGKAPKLLIYLASTLASGVPSRFSGSGSGAEFTLTISSLQPDDFATYYCQNVYLASTNGANFGQGTKLTVLGGGGGSGGGGSGGGGSGGGGSEVQLVESGGGLVQPGGSLRLSCTASGFSLTDYYYMTWVRQAPGKGLEWVGFIDPDDDPYYATWAKGRFTISRDNSKNTLYLQMNSLRAEDTAVYYCAGGDHNSGWGLDIWGQGTLVTVSSGGGGSGGGGSGGGGSGGGGSGGGGSSDTGRPFVEMYSEIPEIIHMTEGRELVIPCRVTSPNITVTLKKFPLDTLIPDGKRIIWDSRKGFIISNATYKEIGLLTCEATVNGHLYKTNYLTHRQTNTIIDVVLSPSHGIELSVGEKLVLNCTARTELNVGIDFNWEYPSSKHQHKKLVNRDLKTQSGSEMKKFLSTLTIDGVTRSDQGLYTCAASSGLMTKKNSTFVRVHEK

SEQ ID NO: 22 - DNA, 1443 bp, synthetic construct
  source 1..1443: mol_type = other DNA
gagatcgtgatgacccagagccctagcacactgagcgcctctgtgggagatagagtgatcatcacctgtcaggcctctgagatcatccacagctggctggcttggtaccagcaaaagcctgggaaggcccctaaactgctgatctatctcgctagcacactggcctctggagtccccagccggtttagcggaagcggctctggcgccgaattcaccctgacaatcagcagcctgcaacccgatgactttgccacatactactgtcagaacgtgtacctggctagcaccaacggcgccaacttcggccagggcacaaagctgaccgtgcttggaggcggcggcggctccggcggaggcggaagcggcggcggcggcagcggcgggggcggcagcgaggtgcagctggtggagtcgggcggcggcctggtgcagccaggaggttctctgaggctgagctgcaccgcaagcggcttcagcctgaccgactactactatatgacatgggtcagacaggcccctggaaagggcctggaatgggtcggatttatcgaccctgacgacgatccttactacgccacttgggccaagggcagatttaccatttccagagataactctaagaacaccctgtacctgcaaatgaacagcctgcgcgccgaggatacagccgtgtactactgcgcaggcggcgaccataattcaggatggggcctggatatctggggccagggcacgctggtgaccgtgtcctccggcggaggaggctctggcggaggcggcagcggcggcggcggctccggcggcggcggcagcggcggtggcggcagcagcgacaccggccggcctttcgtggaaatgtacagcgagatccccgagatcatccacatgaccgagggcagagagctggtgatcccctgccgggtgaccagccctaacatcaccgtgaccctgaagaaattccccctggacacactgatccccgatggaaaaagaatcatctgggacagcagaaagggcttcatcatttctaatgccacatacaaggaaatcggcctgctgacttgtgaagccaccgtgaacggccacctgtacaagaccaactacctgactcatagacaaacaaacacaatcatcgacgtggtgctgagcccttctcatggcatcgagctctctgtgggcgagaagctggtgctgaattgcaccgctcgcaccgagctgaacgtgggaatcgacttcaactgggagtacccttcttctaagcaccagcacaagaagctggtgaaccgggacctgaagacccagagcggcagcgaaatgaaaaagttcctgtccacactgaccattgacggcgtgacaagaagcgaccagggcctgtatacatgtgccgcctcttctgggctgatgaccaagaagaacagcaccttcgtgcgggtgcacgagaag

SEQ ID NO: 23 - DNA, 5839 bp, synthetic construct
  source 1..5839: mol_type = other DNA
ggccgcgttgctggcgtttttccataggctccgcccccctgacgagcatcacaaaaatcgacgctcaagtcagaggtggcgaaacccgacaggactataaagataccaggcgtttccccctggaagctccctcgtgcgctctcctgttccgaccctgccgcttaccggatacctgtccgcctttctcccttcgggaagcgtggcgctttctcatagctcacgctgtaggtatctcagttcggtgtaggtcgttcgctccaagctgggctgtgtgcacgaaccccccgttcagcccgaccgctgcgccttatccggtaactatcgtcttgagtccaacccggtaagacacgacttatcgccactggcagcagccactggtaacaggattagcagagcgaggtatgtaggcggtgctacagagttcttgaagtggtggcctaactacggctacactagaagaacagtatttggtatctgcgctctgctgaagccagttaccttcggaaaaagagttggtagctcttgatccggcaaacaaaccaccgctggtagcggtggtttttttgtttgcaagcagcagattacgcgcagaaaaaaaggatctcaagaagatcctttgatcttttctacggggtctgacgctcagtggaacgaaaactcacgttaagggattttggtcatgaagcgcttttgaagctcggatccgaacaaacgacccaacacccgtgcgttttattctgtctttttattgccgatcccctcagaagaactcgtcaagaaggcgatagaaggcgatgcgctgcgaatcgggagcggcgataccgtaaagcacgaggaagcggtcagcccattcgccgccaagctcttcagcaatatcacgggtagccaacgctatgtcctgatagcggtccgccacacccagccggccacagtcgatgaatccagaaaagcggccattttccaccatgatattcggcaagcaggcatcgccatgggtcacgacgagatcctcgccgtcgggcatgctcgccttgagcctggcgaacagttcggctggcgcgagcccctgatgctcttcgtccagatcatcctgatcgacaagaccggcttccatccgagtacgtgctcgctcgatgcgatgtttcgcttggtggtcgaatgggcaggtagccggatcaagcgtatgcagccgccgcattgcatcagccatgatggatactttctcggcaggagcaaggtgagatgacaggagatcctgccccggcacttcgcccaatagcagccagtcccttcccgcttcagtgacaacgtcgagcacagctgcgcaaggaacgcccgtcgtggccagccacgatagccgcgctgcctcgtcttgcagttcattcagggcaccggacaggtcggtcttgacaaaaagaaccgggcgcccctgcgctgacagccggaacacggcggcatcagagcagccgattgtctgttgtgcccagtcatagccgaatagcctctccacccaagcggccggagaacctgcgtgcaatccatcttgttcaatcatgcgaaacgatcctcatcctgtctcttgatcagagcttgatcccctgcgccatcagatccttggcggcaagaaagccatccagtttactttgcagggcttcccaaccttaccagaggcctgcgccgcggccagctggctagcaattcccgggttaactctagagacattgattattgactagttattaatagtaatcaattacggggtcattagttcatagcccatatatggagttccgcgttacataacttacggtaaatggcccgcctggctgaccgcccaacgacccccgcccattgacgtcaataatgacgtatgttcccatagtaacgccaatagggactttccattgacgtcaatgggtggagtatttacggtaaactgcccacttggcagtacatcaagtgtatcatatgccaagtacgccccctattgacgtcaatgacggtaaatggcccgcctggcattatgcccagtacatgaccttatgggactttcctacttggcagtacatctacgtattagtcatcgctattaccatggtgatgcggttttggcagtacatcaatgggcgtggatagcggtttgactcacggggatttccaagtctccaccccattgacgtcaatgggagtttgttttggcaccaaaatcaacgggactttccaaaatgtcgtaacaactccgccccattgacgcaaatgggcggtaggcgtgtacggtgggaggtctatataagcagagctcgtttagtgaaccggggtctctctggttagaccagatctgagcctgggagctctctggctaactagggaacccactgcttaagcctcaataaagcttgccttgagtgcttcaagtagtgtgtgcccgtctgttgtgtgactctggtaactagagatccctcagacccttttagtcagtgtggaaaatctctagcagtggcgcccgaacagggacttgaaagcgaaagggaaaccagaggagctctctcgacgcaggactcggcttgctgaagcgcgcacggcaagaggcgaggggcggcgactggtgagtacgccaaaaattttgactagcggaggctagaaggagagagatgggtgcgagagcgtcagtattaagcgggggagaattagatcgcgatgggaaaaaattcggttaaggccagggggaaagaaaaaatataaattaaaacatatagtatgggcaagcagggagctagaacgattcgcagttaatcctggcctgttagaaacatcagaaggctgtagacaaatactgggacagctacaaccatcccttcagacaggatcagaagaacttagatcattatataatacagtagcaaccctctattgtgtgcatcaaaggatagagataaaagacaccaaggaagctttagacaagatagaggaagagcaaaacaaaagtaagaccaccgcacagcaagcggccgctgatcttcagacctggaggaggagatatgagggacaattggagaagtgaattatataaatataaagtagtaaaaattgaaccattaggagtagcacccaccaaggcaaagagaagagtggtgcagagagaaaaaagagcagtgggaataggagctttgttccttgggttcttgggagcagcaggaagcactatgggcgcagcgtcaatgacgctgacggtacaggccagacaattattgtctggtatagtgcagcagcagaacaatttgctgagggctattgaggcgcaacagcatctgttgcaactcacagtctggggcatcaagcagctccaggcaagaatcctggctgtggaaagatacctaaaggatcaacagctcctggggatttggggttgctctggaaaactcatttgcaccactgctgtgccttggaatgctagttggagtaataaatctctggaacagatttggaatcacacgacctggatggagtgggacagagaaattaacaattacacaagcttaatacactccttaattgaagaatcgcaaaaccagcaagaaaagaatgaacaagaattattggaattagataaatgggcaagtttgtggaattggtttaacataacaaattggctgtggtatataaaattattcataatgatagtaggaggcttggtaggtttaagaatagtttttgctgtactttctatagtgaatagagttaggcagggatattcaccattatcgtttcagacccacctcccaaccccgaggggacccgacaggcccgaaggaatagaagaagaaggtggagagagagacagagacagatccattcgattagtgaacggatctcgacggtatcggttaacttttaaaagaaaaggggggattggggggtacagtgcaggggaaagaatagtagacataatagcaacagacatacaaactaaagaattacaaaaacaaattacaaaaattcaaaattttatcgatcacgagactagcctcgagaagcttgatatccgtcgacacgcgtgacaatcaacctctggattacaaaatttgtgaaagattgactggtattcttaactatgttgctccttttacgctatgtggatacgctgctttaatgcctttgtatcatgctattgcttcccgtatggctttcattttctcctccttgtataaatcctggttgctgtctctttatgaggagttgtggcccgttgtcaggcaacgtggcgtggtgtgcactgtgtttgctgacgcaacccccactggttggggcattgccaccacctgtcagctcctttccgggactttcgctttccccctccctattgccacggcggaactcatcgccgcctgccttgcccgctgctggacaggggctcggctgttgggcactgacaattccgtggtgttgtcggggaagctgacgtcctttccatggctgctcgcctgtgttgccacctggattctgcgcgggacgtccttctgctacgtcccttcggccctcaatccagcggaccttccttcccgcggcctgctgccggctctgcggcctcttccgcgtcttcgccttcgccctcagacgagtcggatctccctttgggccgcctccccgcctggaattcgagctcggtacctttaagaccaatgacttacaaggcagctgtagatcttagccactttttaaaagaaaaggggggactggaagggctaattcactcccaacgaagacaagatctgctttttgcttgtactgggtctctctggttagaccagatctgagcctgggagctctctggctaactagggaacccactgcttaagcctcaataaagcttgccttgagtgcttcaagtagtgtgtgcccgtctgttgtgtgactctggtaactagagatccctcagacccttttagtcagtgtggaaaatctctagcagtagtagttcatgtcatcttattattcagtatttataacttgcaaagaaatgaatatcagagagtgagaggaacttgtttattgcagcttataatggttacaaataaagcaatagcatcacaaatttcacaaataaagcatttttttcactgcattctagttgtggtttgtccaaactcatcaatgtatcttatcatgtctggctctagctatcccgcccctaactccgcccatcccgcccctaactccgcccagttccgcccattctccgccccatggctgactaattttttttatttatgcagaggccgaggccgcctcggcctctgagctattccagaagtagtgaggaggcttttttggaggccgctagcgtcgaccattacttattgttttagctgtcctcatgaatgtcttttcactacccatttgcttatcctgcatctctcagccttgactccactcagttctcttgcttagagataccacctttcccctgaagtgttccttccatgttttacggcgagatggtttctcctcgcctggccactcagccttagttgtctctgttgtcttatagaggtctacttgaagaaggaaaaacagggggcatggtttgactgtcctgtgagcccttcttccctgcctcccccactcacagtgacccggaatccctcgacatggcagtctagcactagtgcggccgcagatctgcttcctcgctcactgactcgctgcgctcggtcgttcggctgcggcgagcggtatcagctcactcaaaggcggtaatacggttatccacagaatcaggggataacgcaggaaagaacatgtgagcaaaaggccagcaaaaggccaggaaccgtaaaaa

SEQ ID NO: 24 - DNA, 3068 bp, synthetic construct
  source 1..3068: mol_type = other DNA
acatgtgagcaaaaggccagcaaaaggccaggaaccgtaaaaaggccgcgttgctggcgtttttccataggctccgcccccctgacgagcatcacaaaaatcgacgctcaagtcagaggtggcgaaacccgacaggactataaagataccaggcgtttccccctggaagctccctcgtgcgctctcctgttccgaccctgccgcttaccggatacctgtccgcctttctcccttcgggaagcgtggcgctttctcatagctcacgctgtaggtatctcagttcggtgtaggtcgttcgctccaagctgggctgtgtgcacgaaccccccgttcagcccgaccgctgcgccttatccggtaactatcgtcttgagtccaacccggtaagacacgacttatcgccactggcagcagccactggtaacaggattagcagagcgaggtatgtaggcggtgctacagagttcttgaagtggtggcctaactacggctacactagaaggacagtatttggtatctgcgctctgctgaagccagttaccttcggaaaaagagttggtagctcttgatccggcaaacaaaccaccgctggtagcggtggtttttttgtttgcaagcagcagattacgcgcagaaaaaaaggatctcaagaagatcctttgatcttttctacggggtctgacgctcagtggaacgaaaactcacgttaagggattttggtcatgagattatcaaaaaggatcttcacctagatccttttaaattaaaaatgaagttttaaatcaatctaaagtatatatgagtaaacttggtctgacagttaccaatgcttaatcagtgaggcacctatctcagcgatctgtctatttcgttcatccatagttgcctgactccccgtcgtgtagataactacgatacgggagggcttaccatctggccccagtgctgcaatgataccgcgagacccacgctcaccggctccagatttatcagcaataaaccagccagccggaagggccgagcgcagaagtggtcctgcaactttatccgcctccatccagtctattaattgttgccgggaagctagagtaagtagttcgccagttaatagtttgcgcaacgttgttgccattgctacaggcatcgtggtgtcacgctcgtcgtttggtatggcttcattcagctccggttcccaacgatcaaggcgagttacatgatcccccatgttgtgcaaaaaagcggttagctccttcggtcctccgatcgttgtcagaagtaagttggccgcagtgttatcactcatggttatggcagcactgcataattctcttactgtcatgccatccgtaagatgcttttctgtgactggtgagtactcaaccaagtcattctgagaatagtgtatgcggcgaccgagttgctcttgcccggcgtcaatacgggataataccgcgccacatagcagaactttaaaagtgctcatcattggaaaacgttcttcggggcgaaaactctcaaggatcttaccgctgttgagatccagttcgatgtaacccactcgtgcacccaactgatcttcagcatcttttactttcaccagcgtttctgggtgagcaaaaacaggaaggcaaaatgccgcaaaaaagggaataagggcgacacggaaatgttgaatactcatactcttcctttttcaatattattgaagcatttatcagggttattgtctcatgagcggatacatatttgaatgtatttagaaaaataaacaaataggggttccgcgcacatttccccgaaaagtgccacctgacgtctaagaaaccattattatcatgacattaacctataaaaataggcgtatcacgaggccctttcgtctcgcgcgtttcggtgatgacggtgaaaacctctgacacatgcagctcccggagacggtcacagcttgtctgtaagcggatgccgggagcagacaagcccgtcagggcgcgtcagcgggtgttggcgggtgtcggggctggcttaactatgcggcatcagagcagattgtactgagagtgcaccataaaattgtaaacgttaatattttgttaaaattcgcgttaaatttttgttaaatcagctcattttttaaccaataggccgaaatcggcaaaatcccttataaatcaaaagaatagcccgagatagggttgagtgttgttccagtttggaacaagagtccactattaaagaacgtggactccaacgtcaaagggcgaaaaaccgtctatcagggcgatggcccactacgtgaaccatcacccaaatcaagttttttggggtcgaggtgccgtaaagcactaaatcggaaccctaaagggagcccccgatttagagcttgacggggaaagccggcgaacgtggcgagaaaggaagggaagaaagcgaaaggagcgggcgctagggcgctggcaagtgtagcggtcacgctgcgcgtaaccaccacacccgccgcgcttaatgcgccgctacagggcgcgtactatggttgctttgacgtatgcggtgtgaaataccgcacagatgcgtaaggagaaaataccgcatcaggcgcccctgcaggcagctgcgcgctcgctcgctcactgaggccgcccgggcaaagcccgggcgtcgggcgacctttggtcgcccggcctcagtgagcgagcgagcgcgcagagagggagtggccaactccatcactaggggttcctacgcgtgtcgacgtttatttgtgaaatttgtgatgctattgctttatttgtaaccatctagctttatttgtgaaatttgtgatgctattgctttatttgtaaccattataagctgcaataaacaagttaacaacaacaattgcattcattttatgtttcaggttcagggggagatgtgggaggttttttaaagtttaaacaggaacccctagtgatggagttggccactccctctctgcgcgctcgctcgctcactgaggccgggcgaccaaaggtcgcccgacgcccgggcggcctcagtgagcgagcgagcgcgcagctgcctgcagg

SEQ ID NO: 25 - DNA, 3387 bp, synthetic construct
  source 1..3387: mol_type = other DNA
ggccgcgttgctggcgtttttccataggctccgcccccctgacgagcatcacaaaaatcgacgctcaagtcagaggtggcgaaacccgacaggactataaagataccaggcgtttccccctggaagctccctcgtgcgctctcctgttccgaccctgccgcttaccggatacctgtccgcctttctcccttcgggaagcgtggcgctttctcatagctcacgctgtaggtatctcagttcggtgtaggtcgttcgctccaagctgggctgtgtgcacgaaccccccgttcagcccgaccgctgcgccttatccggtaactatcgtcttgagtccaacccggtaagacacgacttatcgccactggcagcagccactggtaacaggattagcagagcgaggtatgtaggcggtgctacagagttcttgaagtggtggcctaactacggctacactagaagaacagtatttggtatctgcgctctgctgaagccagttaccttcggaaaaagagttggtagctcttgatccggcaaacaaaccaccgctggtagcggtggtttttttgtttgcaagcagcagattacgcgcagaaaaaaaggatctcaagaagatcctttgatcttttctacggggtctgacgctcagtggaacgaaaactcacgttaagggattttggtcatgaagcgcttttgaagctcggatccgaacaaacgacccaacacccgtgcgttttattctgtctttttattgccgatcccctcagaagaactcgtcaagaaggcgatagaaggcgatgcgctgcgaatcgggagcggcgataccgtaaagcacgaggaagcggtcagcccattcgccgccaagctcttcagcaatatcacgggtagccaacgctatgtcctgatagcggtccgccacacccagccggccacagtcgatgaatccagaaaagcggccattttccaccatgatattcggcaagcaggcatcgccatgggtcacgacgagatcctcgccgtcgggcatgctcgccttgagcctggcgaacagttcggctggcgcgagcccctgatgctcttcgtccagatcatcctgatcgacaagaccggcttccatccgagtacgtgctcgctcgatgcgatgtttcgcttggtggtcgaatgggcaggtagccggatcaagcgtatgcagccgccgcattgcatcagccatgatggatactttctcggcaggagcaaggtgagatgacaggagatcctgccccggcacttcgcccaatagcagccagtcccttcccgcttcagtgacaacgtcgagcacagctgcgcaaggaacgcccgtcgtggccagccacgatagccgcgctgcctcgtcttgcagttcattcagggcaccggacaggtcggtcttgacaaaaagaaccgggcgcccctgcgctgacagccggaacacggcggcatcagagcagccgattgtctgttgtgcccagtcatagccgaatagcctctccacccaagcggccggagaacctgcgtgcaatccatcttgttcaatcatgcgaaacgatcctcatcctgtctcttgatcagagcttgatcccctgcgccatcagatccttggcggcaagaaagccatccagtttactttgcagggcttcccaaccttaccagaggcctgcgccgcggccagctggctagcaattcccgggttaactctagagaatgtagtcttatgcaatactcttgtagtcttgcaacatggtaacgatgagttagcaacatgccttacaaggagagaaaaagcaccgtgcatgccgattggtggaagtaaggtggtacgatcgtgccttattaggaaggcaacagacgggtctgacatggattggacgaaccactgaattccgcattgcagagatattgtatttaagtgcctagctcgatacaataaacgccatttgaccattcaccacattggtgtgcacctccaagctcgagctcgtttagtgaaccgtcagatcgcctggagacgccatccacgctgttttgacctccatagaagacaccgggaccgatccagcctcccctcgaagctagtcgattaggcatctcctatggcaggaagaagcggagacagcgacgaagacctcctcaaggcagtcagactcatcaagtttctctatcaaagcaacccacctcccaatcccgaggggacccgacaggcccgaaggaatagaagaagaaggtggagagagagacagagacagatccattcgattagtgaacggatccttagcacttatctgggacgatctgcggagcctgtgcctcttcagctaccaccgcttgagagacttactcttgattgtaacgaggattgtggaacttctgggacgcagggggtgggaagccctcaaatattggtggaatctcctacaatattggagtcaggagctaaagaatagtgctgttagcttgctcaatgccacagctatagcagtagctgaggggacagatagggttatagaagtagtacaagaagcttggcactggccgtcgttttacaacgtcgtgatctgagcctgggagatctctggctaactagggaacccactgcttaagcctcaataaagcttgccttgagtgcttcaagtagtgtgtgcccgtctgttgtgtgactctggtaactagagatcaggaaaaccctggcgttacccaacttaatcgccttgcagcacatccccctttcgccagctggcgtaatagcgaagaggcccgcaccgatcgcccttcccaacagttgcgcagcctgaatggcgaatggcgcctgatgcggtattttctccttacgcatctgtgcggtatttcacaccgcatacgtcaaagcaaccatagtgtcgaccattacttattgttttagctgtcctcatgaatgtcttttcactacccatttgcttatcctgcatctctcagccttgactccactcagttctcttgcttagagataccacctttcccctgaagtgttccttccatgttttacggcgagatggtttctcctcgcctggccactcagccttagttgtctctgttgtcttatagaggtctacttgaagaaggaaaaacagggggcatggtttgactgtcctgtgagcccttcttccctgcctcccccactcacagtgacccggaatccctcgacatggcagtctagcactagtgcggccgcagatctgcttcctcgctcactgactcgctgcgctcggtcgttcggctgcggcgagcggtatcagctcactcaaaggcggtaatacggttatccacagaatcaggggataacgcaggaaagaacatgtgagcaaaaggccagcaaaaggccaggaaccgtaaaaa

SEQ ID NO: 26 - DNA, 9171 bp, synthetic construct
  source 1..9171: mol_type = other DNA
ggccgcgttgctggcgtttttccataggctccgcccccctgacgagcatcacaaaaatcgacgctcaagtcagaggtggcgaaacccgacaggactataaagataccaggcgtttccccctggaagctccctcgtgcgctctcctgttccgaccctgccgcttaccggatacctgtccgcctttctcccttcgggaagcgtggcgctttctcatagctcacgctgtaggtatctcagttcggtgtaggtcgttcgctccaagctgggctgtgtgcacgaaccccccgttcagcccgaccgctgcgccttatccggtaactatcgtcttgagtccaacccggtaagacacgacttatcgccactggcagcagccactggtaacaggattagcagagcgaggtatgtaggcggtgctacagagttcttgaagtggtggcctaactacggctacactagaagaacagtatttggtatctgcgctctgctgaagccagttaccttcggaaaaagagttggtagctcttgatccggcaaacaaaccaccgctggtagcggtggtttttttgtttgcaagcagcagattacgcgcagaaaaaaaggatctcaagaagatcctttgatcttttctacggggtctgacgctcagtggaacgaaaactcacgttaagggattttggtcatgaagcgcttttgaagctcggatccgaacaaacgacccaacacccgtgcgttttattctgtctttttattgccgatcccctcagaagaactcgtcaagaaggcgatagaaggcgatgcgctgcgaatcgggagcggcgataccgtaaagcacgaggaagcggtcagcccattcgccgccaagctcttcagcaatatcacgggtagccaacgctatgtcctgatagcggtccgccacacccagccggccacagtcgatgaatccagaaaagcggccattttccaccatgatattcggcaagcaggcatcgccatgggtcacgacgagatcctcgccgtcgggcatgctcgccttgagcctggcgaacagttcggctggcgcgagcccctgatgctcttcgtccagatcatcctgatcgacaagaccggcttccatccgagtacgtgctcgctcgatgcgatgtttcgcttggtggtcgaatgggcaggtagccggatcaagcgtatgcagccgccgcattgcatcagccatgatggatactttctcggcaggagcaaggtgagatgacaggagatcctgccccggcacttcgcccaatagcagccagtcccttcccgcttcagtgacaacgtcgagcacagctgcgcaaggaacgcccgtcgtggccagccacgatagccgcgctgcctcgtcttgcagttcattcagggcaccggacaggtcggtcttgacaaaaagaaccgggcgcccctgcgctgacagccggaacacggcggcatcagagcagccgattgtctgttgtgcccagtcatagccgaatagcctctccacccaagcggccggagaacctgcgtgcaatccatcttgttcaatcatgcgaaacgatcctcatcctgtctcttgatcagagcttgatcccctgcgccatcagatccttggcggcaagaaagccatccagtttactttgcagggcttcccaaccttaccagaggcctgcgccgcggccagctggctagcaattcccgggttaactctagagacattgattattgactagttattaatagtaatcaattacggggtcattagttcatagcccatatatggagttccgcgttacataacttacggtaaatggcccgcctggctgaccgcccaacgacccccgcccattgacgtcaataatgacgtatgttcccatagtaacgccaatagggactttccattgacgtcaatgggtggagtatttacggtaaactgcccacttggcagtacatcaagtgtatcatatgccaagtacgccccctattgacgtcaatgacggtaaatggcccgcctggcattatgcccagtacatgaccttatgggactttcctacttggcagtacatctacgtattagtcatcgctattaccatggtgatgcggttttggcagtacatcaatgggcgtggatagcggtttgactcacggggatttccaagtctccaccccattgacgtcaatgggagtttgttttggcaccaaaatcaacgggactttccaaaatgtcgtaacaactccgccccattgacgcaaatgggcggtaggcgtgtacggtgggaggtctatataagcagagctcgtttagtgaaccgtcagatcgcctggagacgccatccacgctgttttgacctccatagaagacaccgggaccgatccagcctcccctcgaagcttacatgtggtaccgagctcggatcctgagaacttcagggtgagtctatgggacccttgatgttttctttccccttcttttctatggttaagttcatgtcataggaaggggagaagtaacagggtacacatattgaccaaatcagggtaattttgcatttgtaattttaaaaaatgctttcttcttttaatatacttttttgtttatcttatttctaatactttccctaatctctttctttcagggcaataatgatacaatgtatcatgcctctttgcaccattctaaagaataacagtgataatttctgggttaaggcaatagcaatatttctgcatataaatatttctgcatataaattgtaactgatgtaagaggtttcatattgctaatagcagctacaatccagctaccattctgcttttattttatggttgggataaggctggattattctgagtccaagctaggcccttttgctaatcatgttcatacctcttatcttcctcccacagctcctgggcaacgtgctggtctgtgtgctggcccatcactttggcaaagcacgtgagatctgaattcgagatctgccgccgccatgggtgcgagagcgtcagtattaagcgggggagaattagatcgatgggaaaaaattcggttaaggccagggggaaagaaaaaatataaattaaaacatatagtatgggcaagcagggagctagaacgattcgcagttaatcctggcctgttagaaacatcagaaggctgtagacaaatactgggacagctacaaccatcccttcagacaggatcagaagaacttagatcattatataatacagtagcaaccctctattgtgtgcatcaaaggatagagataaaagacaccaaggaagctttagacaagatagaggaagagcaaaacaaaagtaagaaaaaagcacagcaagcagcagctgacacaggacacagcaatcaggtcagccaaaattaccctatagtgcagaacatccaggggcaaatggtacatcaggccatatcacctagaactttaaatgcatgggtaaaagtagtagaagagaaggctttcagcccagaagtgatacccatgttttcagcattatcagaaggagccaccccacaagatttaaacaccatgctaaacacagtggggggacatcaagcagccatgcaaatgttaaaagagaccatcaatgaggaagctgcagaatgggatagagtgcatccagtgcatgcagggcctattgcaccaggccagatgagagaaccaaggggatcagacatcgctggaactactagtacccttcaggaacaaataggatggatgacacataatccacctatcccagtaggagaaatctataaaagatggataatcctgggattaaataaaatagtaagaatgtatagccctaccagcattctggacataagacaaggaccaaaggaaccctttagagactatgtagaccgattctataaaactctaagagccgagcaagcttcacaagaggtaaaaaattggatgacagaaaccttgttggtccaaaatgcgaacccagattgtaagactattttaaaagcattgggaccaggagcgacactagaagaaatgatgacagcatgtcagggagtggggggacccggccataaagcaagagttttggctgaagcaatgagccaagtaacaaatccagctaccataatgatacagaaaggcaattttaggaaccaaagaaagactgttaagtgtttcaattgtggcaaagaagggcacatagccaaaaattgcagggcccctaggaaaaagggctgttggaaatgtggaaaggaaggacaccaaatgaaagattgtactgagagacaggctaattttttagggaagatctggccttcccacaagggaaggccagggaattttcttcagagcagaccagagccaacagccccaccagaagagagcttcaggtttggggaagagacaacaactccctctcagaagcaggagccgatagacaaggaactgtatcctttagcttccctcagatcactctttggcagcgacccctcgtcacaataaagataggggggcaattaaaggaagctctattagatactggtgctgacgacacagtattagaagaaatgaatttgccaggaagatggaaaccaaaaatgatagggggaattggaggttttatcaaagtaagacagtatgatcagatactcatagaaatctgcggacataaagctataggtacagtattagtaggacctacacctgtcaacataattggaagaaatctgttgactcagattggctgcactttaaattttcccattagtcctattgagactgtaccagtaaaattaaagccaggaatggatggcccaaaagttaaacaatggccattgacagaagaaaaaataaaagcattagtagaaatttgtacagaaatggaaaaggaaggaaaaatttcaaaaattgggcctgaaaatccatacaatactccagtatttgccataaagaaaaaagacagtactaaatggagaaaattagtagatttcagagaacttaataagagaactcaagatttctgggaagttcaattaggaataccacatcctgcagggttaaaacagaaaaaatcagtaacagtactggatgtgggcgatgcatatttttcagttcccttagataaagacttcaggaagtatactgcatttaccatacctagtataaacaatgagacaccagggattagatatcagtacaatgtgcttccacagggatggaaaggatcaccagcaatattccagtgtagcatgacaaaaatcttagagccttttagaaaacaaaatccagacatagtcatctatcaatacatggatgatttgtatgtaggatctgacttagaaatagggcagcatagaacaaaaatagaggaactgagacaacatctgttgaggtggggatttaccacaccagacaaaaaacatcagaaagaacctccattcctttggatgggttatgaactccatcctgataaatggacagtacagcctatagtgctgccagaaaaggacagctggactgtcaatgacatacagaaattagtgggaaaattgaattgggcaagtcagatttatgcagggattaaagtaaggcaattatgtaaacttcttaggggaaccaaagcactaacagaagtagtaccactaacagaagaagcagagctagaactggcagaaaacagggagattctaaaagaaccggtacatggagtgtattatgacccatcaaaagacttaatagcagaaatacagaagcaggggcaaggccaatggacatatcaaatttatcaagagccatttaaaaatctgaaaacaggaaagtatgcaagaatgaagggtgcccacactaatgatgtgaaacaattaacagaggcagtacaaaaaatagccacagaaagcatagtaatatggggaaagactcctaaatttaaattacccatacaaaaggaaacatgggaagcatggtggacagagtattggcaagccacctggattcctgagtgggagtttgtcaatacccctcccttagtgaagttatggtaccagttagagaaagaacccataataggagcagaaactttctatgtagatggggcagccaatagggaaactaaattaggaaaagcaggatatgtaactgacagaggaagacaaaaagttgtccccctaacggacacaacaaatcagaagactgagttacaagcaattcatctagctttgcaggattcgggattagaagtaaacatagtgacagactcacaatatgcattgggaatcattcaagcacaaccagataagagtgaatcagagttagtcagtcaaataatagagcagttaataaaaaaggaaaaagtctacctggcatgggtaccagcacacaaaggaattggaggaaatgaacaagtagataaattggtcagtgctggaatcaggaaagtactatttttagatggaatagataaggcccaagaagaacatgagaaatatcacagtaattggagagcaatggctagtgattttaacctaccacctgtagtagcaaaagaaatagtagccagctgtgataaatgtcagctaaaaggggaagccatgcatggacaagtagactgtagcccaggaatatggcagctagattgtacacatttagaaggaaaagttatcttggtagcagttcatgtagccagtggatatatagaagcagaagtaattccagcagagacagggcaagaaacagcatacttcctcttaaaattagcaggaagatggccagtaaaaacagtacatacagacaatggcagcaatttcaccagtactacagttaaggccgcctgttggtgggcggggatcaagcaggaatttggcattccctacaatccgcagtcacaaggagtaatagaatctatgaataaagaattaaagaaaattataggacaggtaagagatcaggctgaacatcttaaaacagcagtacaaatggcagtattcatccacaattttaaaagaaaaggggggattggggggtacagtgcaggggaaagaatagtagacataatagcaacagacatacaaactaaagaattacaaaaacaaattacaaaaattcaaaattttcgggtttattacagggacagcagagatccagtttggaaaggaccagcaaagctcctctggaaaggtgaaggggcagtagtaatacaagataatagtgacataaaagtagtgccaagaagaaaagcaaagatcatcagggattatggaaaacagatggcaggtgatgattgtgtggcaagtagacaggatgaggattaacacatggaattccggagcggccgcaggagctttgttccttgggttcttgggagcagcaggaagcactatgggcgcagcgtcaatgacgctgacggtacaggccagacaattattgtctggtatagtgcagcagcagaacaatttgctgagggctattgaggcgcaacagcatctgttgcaactcacagtctggggcatcaagcagctccaggcaagaatcctggctgtggaaagatacctaaaggatcaacagctcctggggatttggggttgctctggaaaactcatttgcaccactgctgtgccttggaatgctagttggagtaataaatctctggaacagatttggaatcacacgacctggatggagtgggacagagaaattaacaattacacaagcttccgcggaattcaccccaccagtgcaggctgcctatcagaaagtggtggctggtgtggctaatgccctggcccacaagtatcactaagctcgctttcttgctgtccaatttctattaaaggttcctttgttccctaagtccaactactaaactgggggatattatgaagggccttgagcatctggattctgcctaataaaaaacatttattttcattgcaatgatgtatttaaattatttctgaatattttactaaaaagggaatgtgggaggtcagtgcatttaaaacataaagaaatgaagagctagttcaaaccttgggaaaatacactatatcttaaactccatgaaagaaggtgaggctgcaaacagctaatgcacattggcaacagcccctgatgcctatgccttattcatccctcagaaaaggattcaagtagaggcttgatttggaggttaaagttttgctatgctgtattttacattacttattgttttagctgtcctcatgaatgtcttttcactacccatttgcttatcctgcatctctcagccttgactccactcagttctcttgcttagagataccacctttcccctgaagtgttccttccatgttttacggcgagatggtttctcctcgcctggccactcagccttagttgtctctgttgtcttatagaggtctacttgaagaaggaaaaacagggggcatggtttgactgtcctgtgagcccttcttccctgcctcccccactcacagtgacccggaatccctcgacatggcagtctagcactagtgcggccgcagatctgcttcctcgctcactgactcgctgcgctcggtcgttcggctgcggcgagcggtatcagctcactcaaaggcggtaatacggttatccacagaatcaggggataacgcaggaaagaacatgtgagcaaaaggccagcaaaaggccaggaaccgtaaaaagtcgaccattacttattgttttagctgtcctcatgaatgtcttttcactacccatttgcttatcctgcatctctcagccttgactccactcagttctcttgcttagagataccacctttcccctgaagtgttccttccatgttttacggcgagatggtttctcctcgcctggccactcagccttagttgtctctgttgtcttatagaggtctacttgaagaaggaaaaacagggggcatggtttgactgtcctgtgagcccttcttccctgcctcccccactcacagtgacccggaatccctcgacatggcagtctagcactagtgcggccgcagatctgcttcctcgctcactgactcgctgcgctcggtcgttcggctgcggcgagcggtatcagctcactcaaaggcggtaatacggttatccacagaatcaggggataacgcaggaaagaacatgtgagcaaaaggccagcaaaaggccaggaaccgtaaaaa

SEQ ID NO: 27 - DNA, 5612 bp, synthetic construct
  source 1..5612: mol_type = other DNA
ggccgcgttgctggcgtttttccataggctccgcccccctgacgagcatcacaaaaatcgacgctcaagtcagaggtggcgaaacccgacaggactataaagataccaggcgtttccccctggaagctccctcgtgcgctctcctgttccgaccctgccgcttaccggatacctgtccgcctttctcccttcgggaagcgtggcgctttctcatagctcacgctgtaggtatctcagttcggtgtaggtcgttcgctccaagctgggctgtgtgcacgaaccccccgttcagcccgaccgctgcgccttatccggtaactatcgtcttgagtccaacccggtaagacacgacttatcgccactggcagcagccactggtaacaggattagcagagcgaggtatgtaggcggtgctacagagttcttgaagtggtggcctaactacggctacactagaagaacagtatttggtatctgcgctctgctgaagccagttaccttcggaaaaagagttggtagctcttgatccggcaaacaaaccaccgctggtagcggtggtttttttgtttgcaagcagcagattacgcgcagaaaaaaaggatctcaagaagatcctttgatcttttctacggggtctgacgctcagtggaacgaaaactcacgttaagggattttggtcatgaagcgcttttgaagctcggatccgaacaaacgacccaacacccgtgcgttttattctgtctttttattgccgatcccctcagaagaactcgtcaagaaggcgatagaaggcgatgcgctgcgaatcgggagcggcgataccgtaaagcacgaggaagcggtcagcccattcgccgccaagctcttcagcaatatcacgggtagccaacgctatgtcctgatagcggtccgccacacccagccggccacagtcgatgaatccagaaaagcggccattttccaccatgatattcggcaagcaggcatcgccatgggtcacgacgagatcctcgccgtcgggcatgctcgccttgagcctggcgaacagttcggctggcgcgagcccctgatgctcttcgtccagatcatcctgatcgacaagaccggcttccatccgagtacgtgctcgctcgatgcgatgtttcgcttggtggtcgaatgggcaggtagccggatcaagcgtatgcagccgccgcattgcatcagccatgatggatactttctcggcaggagcaaggtgagatgacaggagatcctgccccggcacttcgcccaatagcagccagtcccttcccgcttcagtgacaacgtcgagcacagctgcgcaaggaacgcccgtcgtggccagccacgatagccgcgctgcctcgtcttgcagttcattcagggcaccggacaggtcggtcttgacaaaaagaaccgggcgcccctgcgctgacagccggaacacggcggcatcagagcagccgattgtctgttgtgcccagtcatagccgaatagcctctccacccaagcggccggagaacctgcgtgcaatccatcttgttcaatcatgcgaaacgatcctcatcctgtctcttgatcagagcttgatcccctgcgccatcagatccttggcggcaagaaagccatccagtttactttgcagggcttcccaaccttaccagaggcctgcgccgcggccagctggctagcaattcccgggttaactctagagacattgattattgactagttattaatagtaatcaattacggggtcattagttcatagcccatatatggagttccgcgttacataacttacggtaaatggcccgcctggctgaccgcccaacgacccccgcccattgacgtcaataatgacgtatgttcccatagtaacgccaatagggactttccattgacgtcaatgggtggagtatttacggtaaactgcccacttggcagtacatcaagtgtatcatatgccaagtacgccccctattgacgtcaatgacggtaaatggcccgcctggcattatgcccagtacatgaccttatgggactttcctacttggcagtacatctacgtattagtcatcgctattaccatggtgatgcggttttggcagtacatcaatgggcgtggatagcggtttgactcacggggatttccaagtctccaccccattgacgtcaatgggagtttgttttggcaccaaaatcaacgggactttccaaaatgtcgtaacaactccgccccattgacgcaaatgggcggtaggcgtgtacggtgggaggtctatataagcagagctcgtttagtgaaccgtcagatcgcctggagacgccatccacgctgttttgacctccatagaagacaccgggaccgatccagcctcccctcgaagcttacatgtggtaccgagctcggatcctgagaacttcagggtgagtctatgggacccttgatgttttctttccccttcttttctatggttaagttcatgtcataggaaggggagaagtaacagggtacacatattgaccaaatcagggtaattttgcatttgtaattttaaaaaatgctttcttcttttaatatacttttttgtttatcttatttctaatactttccctaatctctttctttcagggcaataatgatacaatgtatcatgcctctttgcaccattctaaagaataacagtgataatttctgggttaaggcaatagcaatatttctgcatataaatatttctgcatataaattgtaactgatgtaagaggtttcatattgctaatagcagctacaatccagctaccattctgcttttattttatggttgggataaggctggattattctgagtccaagctaggcccttttgctaatcatgttcatacctcttatcttcctcccacagctcctgggcaacgtgctggtctgtgtgctggcccatcactttggcaaagcacgtgagatctgaattctgacactatgaagtgccttttgtacttagcctttttattcattggggtgaattgcaagttcaccatagtttttccacacaaccaaaaaggaaactggaaaaatgttccttctaattaccattattgcccgtcaagctcagatttaaattggcataatgacttaataggcacagccttacaagtcaaaatgcccaagagtcacaaggctattcaagcagacggttggatgtgtcatgcttccaaatgggtcactacttgtgatttccgctggtatggaccgaagtatataacacattccatccgatccttcactccatctgtagaacaatgcaaggaaagcattgaacaaacgaaacaaggaacttggctgaatccaggcttccctcctcaaagttgtggatatgcaactgtgacggatgccgaagcagtgattgtccaggtgactcctcaccatgtgctggttgatgaatacacaggagaatgggttgattcacagttcatcaacggaaaatgcagcaattacatatgccccactgtccataactctacaacctggcattctgactataaggtcaaagggctatgtgattctaacctcatttccatggacatcaccttcttctcagaggacggagagctatcatccctgggaaaggagggcacagggttcagaagtaactactttgcttatgaaactggaggcaaggcctgcaaaatgcaatactgcaagcattggggagtcagactcccatcaggtgtctggttcgagatggctgataaggatctctttgctgcagccagattccctgaatgcccagaagggtcaagtatctctgctccatctcagacctcagtggatgtaagtctaattcaggacgttgagaggatcttggattattccctctgccaagaaacctggagcaaaatcagagcgggtcttccaatctctccagtggatctcagctatcttgctcctaaaaacccaggaaccggtcctgctttcaccataatcaatggtaccctaaaatactttgagaccagatacatcagagtcgatattgctgctccaatcctctcaagaatggtcggaatgatcagtggaactaccacagaaagggaactgtgggatgactgggcaccatatgaagacgtggaaattggacccaatggagttctgaggaccagttcaggatataagtttcctttatacatgattggacatggtatgttggactccgatcttcatcttagctcaaaggctcaggtgttcgaacatcctcacattcaagacgctgcttcgcaacttcctgatgatgagagtttattttttggtgatactgggctatccaaaaatccaatcgagcttgtagaaggttggttcagtagttggaaaagctctattgcctcttttttctttatcatagggttaatcattggactattcttggttctccgagttggtatccatctttgcattaaattaaagcacaccaagaaaagacagatttatacagacatagagatgaaccgacttggaaagtaactcaaatcctgcacaacagattcttcatgtttggaccaaatcaacttgtgataccatgctcaaagaggcctcaattatatttgagtttttaatttttatgaaaaaaaaaaaaaaaaacggaattcaccccaccagtgcaggctgcctatcagaaagtggtggctggtgtggctaatgccctggcccacaagtatcactaagctcgctttcttgctgtccaatttctattaaaggttcctttgttccctaagtccaactactaaactgggggatattatgaagggccttgagcatctggattctgcctaataaaaaacatttattttcattgcaatgatgtatttaaattatttctgaatattttactaaaaagggaatgtgggaggtcagtgcatttaaaacataaagaaatgaagagctagttcaaaccttgggaaaatacactatatcttaaactccatgaaagaaggtgaggctgcaaacagctaatgcacattggcaacagcccctgatgcctatgccttattcatccctcagaaaaggattcaagtagaggcttgatttggaggttaaagttttgctatgctgtattttagtcgaccattacttattgttttagctgtcctcatgaatgtcttttcactacccatttgcttatcctgcatctctcagccttgactccactcagttctcttgcttagagataccacctttcccctgaagtgttccttccatgttttacggcgagatggtttctcctcgcctggccactcagccttagttgtctctgttgtcttatagaggtctacttgaagaaggaaaaacagggggcatggtttgactgtcctgtgagcccttcttccctgcctcccccactcacagtgacccggaatccctcgacatggcagtctagcactagtgcggccgcagatctgcttcctcgctcactgactcgctgcgctcggtcgttcggctgcggcgagcggtatcagctcactcaaaggcggtaatacggttatccacagaatcaggggataacgcaggaaagaacatgtgagcaaaaggccagcaaaaggccaggaaccgtaaaaa

SEQ ID NO: 28 - DNA, 812 bp, synthetic construct
  source 1..812: mol_type = other DNA
cgttacataacttacggtaaatggcccgcctggctgaccgcccaacgacccccgcccattgacgtcaataatgacgtatgttcccatagtaacgccaatagggactttccattgacgtcaatgggtggagtatttacggtaaactgcccacttggcagtacatcaagtgtatcatatgccaagtacgccccctattgacgtcaatgacggtaaatggcccgcctggcattatgcccagtacatgaccttatgggactttcctacttggcagtacatctacgtattagtcatcgctattaccatggtcgaggtgagccccacgttctgcttcactctccccatctcccccccctccccacccccaattttgtatttatttattttttaattattttgtgcagcgatgggggcggggggggggggggggcgcgcgccaggcggggcggggcggggcgaggggcggggcggggcgaggcggagaggtgcggcggcagccaatcagagcggcgcgctccgaaagtttccttttatggcgaggcggcggcggcggcggccctataaaaagcgaagcgcgcggcgggcgggagtcgctgcgacgctgccttcgccccgtgccccgctccgccgccgcctcgcgccgcccgccccggctctgactgaccgcgttactcccacaggtgagcgggcgggacggcccttctcctccgggctgtaattagctgagcaagaggtaagggtttaagggatggttggttggtggggtattaatgtttaattacctggagcacctgcctgaaatcactttttttcag

SEQ ID NO: 29 - DNA, 568 bp, synthetic construct
  source 1..568: mol_type = other DNA
tagttattaatagtaatcaattacggggtcattagttcatagcccatatatggagttccgcgttacataacttacggtaaatggcccgcctggctgaccgcccaacgacccccgcccattgacgtcaataatgacgtatgttcccatagtaacgccaatagggactttccattgacgtcaatgggtggagtatttacggtaaactgcccacttggcagtacatcaagtgtatcatatgccaagtacgccccctattgacgtcaatgacggtaaatggcccgcctggcattatgcccagtacatgaccttatgggactttcctacttggcagtacatctacgtattagtcatcgctattaccatggtgatgcggttttggcagtacatcaatgggcgtggatagcggtttgactcacggggatttccaagtctccaccccattgacgtcaatgggagtttgttttggcaccaaaatcaacgggactttccaaaatgtcgtaacaactccgccccattgacgcaaatgggcggtaggcgtgtacggtgggaggtctatataagcagagct

SEQ ID NO: 30 - DNA, 1662 bp, synthetic construct
  source 1..1662: mol_type = other DNA
tagttattaatagtaatcaattacggggtcattagttcatagcccatatatggagttccgcgttacataacttacggtaaatggcccgcctggctgaccgcccaacgacccccgcccattgacgtcaataatgacgtatgttcccatagtaacgccaatagggactttccattgacgtcaatgggtggagtatttacggtaaactgcccacttggcagtacatcaagtgtatcatatgccaagtacgccccctattgacgtcaatgacggtaaatggcccgcctggcattatgcccagtacatgaccttatgggactttcctacttggcagtacatctacgtattagtcatcgctattaccatggtcgaggtgagccccacgttctgcttcactctccccatctcccccccctccccacccccaattttgtatttatttattttttaattattttgtgcagcgatgggggcggggggggggggggggcgcgcgccaggcggggcggggcggggcgaggggcggggcggggcgaggcggagaggtgcggcggcagccaatcagagcggcgcgctccgaaagtttccttttatggcgaggcggcggcggcggcggccctataaaaagcgaagcgcgcggcgggcggggagtcgctgcgacgctgccttcgccccgtgccccgctccgccgccgcctcgcgccgcccgccccggctctgactgaccgcgttactcccacaggtgagcgggcgggacggcccttctcctccgggctgtaattagcgcttggtttaatgacggcttgtttcttttctgtggctgcgtgaaagccttgaggggctccgggagggccctttgtgcggggggagcggctcggggggtgcgtgcgtgtgtgtgtgcgtggggagcgccgcgtgcggctccgcgctgcccggcggctgtgagcgctgcgggcgcggcgcggggctttgtgcgctccgcagtgtgcgcgaggggagcgcggccgggggcggtgccccgcggtgcggggggggctgcgaggggaacaaaggctgcgtgcggggtgtgtgcgtgggggggtgagcagggggtgtgggcgcgtcggtcgggctgcaaccccccctgcacccccctccccgagttgctgagcacggcccggcttcgggtgcggggctccgtacggggcgtggcgcggggctcgccgtgccgggcggggggtggcggcaggtgggggtgccgggcggggcggggccgcctcgggccggggagggctcgggggaggggcgcggcggcccccggagcgccggcggctgtcgaggcgcggcgagccgcagccattgccttttatggtaatcgtgcgagagggcgcagggacttcctttgtcccaaatctgtgcggagccgaaatctgggaggcgccgccgcaccccctctagcgggcgcggggcgaagcggtgcggcgccggcaggaaggaaatgggcggggagggccttcgtgcgtcgccgcgccgccgtccccttctccctctccagcctcggggctgtccgcggggggacggctgccttcgggggggacggggcagggcggggttcggcttctggcgtgtgaccggcggctctagagcctctgctaaccatgttcatgccttcttctttttcctacag

SEQ ID NO: 31 - DNA, 897 bp, synthetic construct
  source 1..897: mol_type = other DNA
ccattgacgtcaataatgacgtatgttcccatagtaacgccaatagggactttccattgacgtcaatgggtggagtatttacggtaaactgcccacttggcagtacatcaagtgtatcatatgccaagtacgccccctattgacgtcaatgacggtaaatggcccgcctggcattatgcccagtacatgaccttatgggactttcctacttggcagtacatctacgtattagtcatcgctattaccatggtcgaggtgagccccacgttctgcttcactctccccatctcccccccctccccacccccaattttgtatttatttattttttaattattttgtgcagcgatgggggcggggggggggggggggcgcgcgccaggcggggcggggcggggcgaggggcggggcggggcgaggcggagaggtgcggcggcagccaatcagagcggcgcgctccgaaagtttccttttatggcgaggcggcggcggcggcggccctataaaaagcgaagcgcgcggcgggcgggagtcgctgcgcgctgccttcgccccgtgccccgctccgccgccgcctcgcgccgcccgccccggctctgactgaccgcgttactcccacaggtgagcgggcgggacggcccttctcctccgggctgtaattagcgcttggtttaatgacggcttgtttcttttctgtggctgcgtgaaagccttgaggggctccgggagggccctttgtgcggggggagcggctcggggctgtccgcggggggacggctgccttcgggggggacggggcagggcggggttcggcttctggcgtgtgaccggcggctctagagcctctgctaaccatgttcatgccttcttctttttcctacagctcctgggcaacgt

SEQ ID NO: 32 - DNA, 764 bp, synthetic construct
  source 1..764: mol_type = other DNA
agatcttcgaaatactctcagagtgccaaacatataccaatggacaagaaggtgaggcagagagcagacaggcattagtgacaagcaaagatatgcagaatttcattctcagcaaatcaaaagtcctcaacctggttggaagaatattggcactgaatggtatcaataaggttgctagagagggttagaggtgcacaatgtgcttccataacattttatacttctccaatcttagcactaatcaaacatggttgaatactttgtttactataactcttacagagttataagatctgtgaagacagggacagggacaatacccatctctgtctggttcataggtggtatgtaatagatatttttaaaaataagtgagttaatgaatgagggtgagaatgaaggcacagaggtattagggggaggtgggccccagagaatggtgccaaggtccagtggggtgactgggatcagctcaggcctgacgctggccactcccacctagctcctttctttctaatctgttctcattctccttgggaaggattgaggtctctggaaaacagccaaacaactgttatgggaacagcaagcccaaataaagccaagcatcagggggatctgagagctgaaagcaacttctgttccccctccctcagctgaaggggtggggaagggctcccaaaaaagccataactccttttaagggatttagaaggcataaaaaggcccctggctgagaacttccttcttcattctgcagttgg

SEQ ID NO: 33 - DNA, 624 bp, synthetic construct
  source 1..624: mol_type = other DNA
gaattctgtcattttactagggtgatgaaattcccaagcaacaccatccttttcagataagggcactgaggctgagagaggagctgaaacctacccggggtcaccacacacaggtggcaaggctgggaccagaaaccaggactgttgactgcagcccggtattcattctttccatagcccacagggctgtcaaagaccccagggcctagtcagaggctcctccttcctggagagttcctggcacagaagttgaagctcagcacagccccctaacccccaactctctctgcaaggcctcaggggtcagaacactggtggagcagatcctttagcctctggattttagggccatggtagagggggtgttgccctaaattccagccctggtctcagcccaacaccctccaagaagaaattagaggggccatggccaggctgtgctagccgttgcttctgagcagattacaagaagggactaagacaaggactcctttgtggaggtcctggcttagggagtcaagtgacggcggctcagcactcacgtgggcagtgccagcctctaagagtgggcaggggcactggccacagagtcccagggagtcccaccagcctagtcgccagacc

SEQ ID NO: 34 - protein, 212 aa, synthetic construct
LGGPSVFLFPPKPKDTLMISRTPEVTCVVVDVSHEDPEVKFNWYVDGVEVHNAKTKPREEQYNSTYRVVSVLTVLHQDWLNGKEYKCKVSNKALPAPIEKTISKAKGQPREPQVYTLPPSRDELTKNQVSLTCLVKGFYPSDIAVEWESNGQPENNYKTTPPVLDSDGSFFLYSKLTVDKSRWQQGNVFSCSVMHEALHNHYTQKSLSLSPG

SEQ ID NO: 35 - DNA, 636 bp, synthetic construct
  source 1..636: mol_type = other DNA
ctgggaggaccaagcgtgttcctgtttccacccaagcccaaggataccctgatgatctccaggaccccagaggtgacatgcgtggtggtggacgtgtctcacgaggatcctgaggtgaagtttaactggtacgtggacggcgtggaggtgcacaatgccaagaccaagcctcgggaggagcagtacaattccacctatagagtggtgtctgtgctgacagtgctgcaccaggattggctgaacggcaaggagtataagtgcaaggtgagcaataaggccctgcctgccccaatcgagaagaccatctccaaggcaaagggacagccaagggagcctcaggtgtacacactgcctccatctcgcgacgagctgaccaagaaccaggtgagcctgacatgtctggtgaagggcttctatccttccgatatcgccgtggagtgggagtctaatggccagccagagaacaattacaagaccacaccccctgtgctggacagcgatggctccttctttctgtattctaagctgaccgtggataagagccggtggcagcagggcaacgtgttttcctgctctgtgatgcacgaggccctgcacaatcactacacccagaagagcctgtccctgtctcccggc

SEQ ID NO: 36 - DNA, 22 bp, synthetic construct
  source 1..22: mol_type = other DNA
ctgttgtgtgactctggtaact

SEQ ID NO: 37 - DNA, 22 bp, synthetic construct
  source 1..22: mol_type = other DNA
aaatctctagcagtggcgcccg

SEQ ID NO: 38 - DNA, 20 bp, synthetic construct
  source 1..20: mol_type = other DNA
ttcgctttcaagtccctgtt

SEQ ID NO: 39 - DNA, 22 bp, synthetic construct
  source 1..22: mol_type = other DNA
gctgtcatctcttgtgggctgt

SEQ ID NO: 40 - DNA, 26 bp, synthetic construct
  source 1..26: mol_type = other DNA
cctgtcatgcccacacaaatctctcc

SEQ ID NO: 41 - DNA, 21 bp, synthetic construct
  source 1..21: mol_type = other DNA
actcatgggagctgctggttc

SEQ ID NO: 42 - DNA, 21 bp, synthetic construct
  source 1..21: mol_type = other DNA
ggaacccctagtgatggagtt

SEQ ID NO: 43 - DNA, 18 bp, synthetic construct
  source 1..18: mol_type = other DNA
cactccctctctgcgcgc

SEQ ID NO: 44 - DNA, 16 bp, synthetic construct
  source 1..16: mol_type = other DNA
cggcctcagtgagcga

SEQ ID NO: 45 - protein, 22 aa, synthetic construct
MDAMKRGLCCVLLLCGAVFVSP

SEQ ID NO: 46 - DNA, 66 bp, synthetic construct
  source 1..66: mol_type = other DNA
atggacgccatgaaaagaggcctgtgctgcgtgctgctgctgtgcggcgccgtgttcgtgtcccct

SEQ ID NO: 47 - protein, 451 aa, synthetic construct
MYRMQLLSCIALSLALVTNSSDTGRPFVEMYSEIPEIIHMTEGRELVIPCRVTSPNITVTLKKFPLDTLIPDGKRIIWDSRKGFIISNATYKEIGLLTCEATVNGHLYKTNYLTHRQTNTIIDVVLSPSHGIELSVGEKLVLNCTARTELNVGIDFNWEYPSSKHQHKKLVNRDLKTQSGSEMKKFLSTLTIDGVTRSDQGLYTCAASSGLMTKKNSTFVRVHEKDKTHTCPPCPAPELLGGPSVFLFPPKPKDTLMISRTPEVTCVVVDVSHEDPEVKFNWYVDGVEVHNAKTKPREEQYNSTYRVVSVLTVLHQDWLNGKEYKCKVSNKALPAPIEKTISKAKGQPREPQVYTLPPSRDELTKNQVSLTCLVKGFYPSDIAVEWESNGQPENNYKTTPPVLDSDGSFFLYSKLTVDKSRWQQGNVFSCSVMHEALHNHYTQKSLSLSPG

SEQ ID NO: 48 - DNA, 1356 bp, synthetic construct
  source 1..1356: mol_type = other DNA
atgtaccggatgcagctgctgtcttgcatcgccctgagcctggccctggtgaccaacagctccgacacaggcagacccttcgtggagatgtattctgagatccctgagatcatccacatgaccgagggcagggagctggtcatcccatgtcgcgtgacaagccccaacatcaccgtgacactgaagaagttccctctggacaccctgatcccagatggcaagcggatcatctgggacagcagaaagggctttatcatctccaatgccacatacaaggagatcggcctgctgacctgcgaggccacagtgaacggccacctgtacaagaccaattatctgacacacagacagaccaacacaatcatcgatgtggtgctgagcccatcccacggcatcgagctgtccgtgggcgagaagctggtgctgaattgtaccgccaggacagagctgaacgtgggcatcgacttcaattgggagtacccctctagcaagcaccagcacaagaagctggtgaacagggatctgaagacccagtctggcagcgagatgaagaagtttctgagcaccctgacaatcgacggagtgacccgctccgatcagggactgtatacatgcgccgcctcctctggcctgatgaccaagaagaattccacattcgtgcgggtgcacgagaaggacaagacccacacatgcccaccttgtccagcaccagagctgctgggaggaccaagcgtgttcctgtttccacccaagcccaaggataccctgatgatctccaggaccccagaggtgacatgcgtggtggtggacgtgtctcacgaggatcctgaggtgaagtttaactggtacgtggacggcgtggaggtgcacaatgccaagaccaagcctcgggaggagcagtacaattccacctatagagtggtgtctgtgctgacagtgctgcaccaggattggctgaacggcaaggagtataagtgcaaggtgagcaataaggccctgcctgccccaatcgagaagaccatctccaaggcaaagggacagccaagggagcctcaggtgtacacactgcctccatctcgcgacgagctgaccaagaaccaggtgagcctgacatgtctggtgaagggcttctatccttccgatatcgccgtggagtgggagtctaatggccagccagagaacaattacaagaccacaccccctgtgctggacagcgatggctccttctttctgtattctaagctgaccgtggataagagccggtggcagcagggcaacgtgttttcctgctctgtgatgcacgaggccctgcacaatcactacacccagaagagcctgtccctgtctcccggctag